European Patent Application EP 4 484 561 A1, published January 1, 2025. Title: EXPRESSION CASSETTE COMBINATIONS AND USES THEREOF. Applicant: CHIGENOVO CO.,LTD. Application EP. The sequence listing filed with the application follows.

SEQUENCE LISTING (44 sequences)

SEQ ID NO: 1 - protein, 2274 aa, Homo sapiens
MGFVRQIQLLLWKNWTLRKRQKIRFVVELVWPLSLFLVLIWLRNANPLYSHHECHFPNKAMPSAGMLPWLQGIFCNVNNPCFQSPTPGESPGIVSNYNNSILARVYRDFQELLMNAPESQHLGRIWTELHILSQFMDTLRTHPERIAGRGIRIRDILKDEETLTLFLIKNIGLSDSVVYLLINSQVRPEQFAHGVPDLALKDIACSEALLERFIIFSQRRGAKTVRYALCSLSQGTLQWIEDTLYANVDFFKLFRVLPTLLDSRSQGINLRSWGGILSDMSPRIQEFIHRPSMQDLLWVTRPLMQNGGPETFTKLMGILSDLLCGYPEGGGSRVLSFNWYEDNNYKAFLGIDSTRKDPIYSYDRRTTSFCNALIQSLESNPLTKIAWRAAKPLLMGKILYTPDSPAARRILKNANSTFEELEHVRKLVKAWEEVGPQIWYFFDNSTQMNMIRDTLGNPTVKDFLNRQLGEEGITAEAILNFLYKGPRESQADDMANFDWRDIFNITDRTLRLVNQYLECLVLDKFESYNDETQLTQRALSLLEENMFWAGVVFPDMYPWTSSLPPHVKYKIRMDIDVVEKTNKIKDRYWDSGPRADPVEDFRYIWGGFAYLQDMVEQGITRSQVQAEAPVGIYLQQMPYPCFVDDSFMIILNRCFPIFMVLAWIYSVSMTVKSIVLEKELRLKETLKNQGVSNAVIWCTWFLDSFSIMSMSIFLLTIFIMHGRILHYSDPFILFLFLLAFSTATIMLCFLLSTFFSKASLAAACSGVIYFTLYLPHILCFAWQDRMTAELKKAVSLLSPVAFGFGTEYLVRFEEQGLGLQWSNIGNSPTEGDEFSFLLSMQMMLLDAAVYGLLAWYLDQVFPGDYGTPLPWYFLLQESYWLGGEGCSTREERALEKTEPLTEETEDPEHPEGIHDSFFEREHPGWVPGVCVKNLVKIFEPCGRPAVDRLNITFYENQITAFLGHNGAGKTTTLSILTGLLPPTSGTVLVGGRDIETSLDAVRQSLGMCPQHNILFHHLTVAEHMLFYAQLKGKSQEEAQLEMEAMLEDTGLHHKRNEEAQDLSGGMQRKLSVAIAFVGDAKVVILDEPTSGVDPYSRRSIWDLLLKYRSGRTIIMSTHHMDEADLLGDRIAIIAQGRLYCSGTPLFLKNCFGTGLYLTLVRKMKNIQSQRKGSEGTCSCSSKGFSTTCPAHVDDLTPEQVLDGDVNELMDVVLHHVPEAKLVECIGQELIFLLPNKNFKHRAYASLFRELEETLADLGLSSFGISDTPLEEIFLKVTEDSDSGPLFAGGAQQKRENVNPRHPCLGPREKAGQTPQDSNVCSPGAPAAHPEGQPPPEPECPGPQLNTGTQLVLQHVQALLVKRFQHTIRSHKDFLAQIVLPATFVFLALMLSIVIPPFGEYPALTLHPWIYGQQYTFFSMDEPGSEQFTVLADVLLNKPGFGNRCLKEGWLPEYPCGNSTPWKTPSVSPNITQLFQKQKWTQVNPSPSCRCSTREKLTMLPECPEGAGGLPPPQRTQRSTEILQDLTDRNISDFLVKTYPALIRSSLKSKFWVNEQRYGGISIGGKLPVVPITGEALVGFLSDLGRIMNVSGGPITREASKEIPDFLKHLETEDNIKVWFNNKGWHALVSFLNVAHNAILRASLPKDRSPEEYGITVISQPLNLTKEQLSEITVLTTSVDAVVAICVIFSMSFVPASFVLYLIQERVNKSKHLQFISGVSPTTYWVTNFLWDIMNYSVSAGLVVGIFIGFQKKAYTSPENLPALVALLLLYGWAVIPMMYPASFLFDVPSTAYVALSCANLFIGINSSAITFILELFENNRTLLRFNAVLRKLLIVFPHFCLGRGLIDLALSQAVTDVYARFGEEHSANPFHWDLIGKNLFAMVVEGVVYFLLTLLVQRHFFLSQWIAEPTKEPIVDEDDDVAEERQRIITGGNKTDILRLHELTKIYPGTSSPAVDRLCVGVRPGECFGLLGVNGAGKTTTFKMLTGDTTVTSGDATVAGKSILTNISEVHQNMGYCPQFDAIDELLTGREHLYLYARLRGVPAEEIEKVANWSIKSLGLTVYADCLAGTYSGGNKRKLSTAIALIGCPPLVLLDEPTTGMDPQARRMLWNVIVSIIREGRAVVLTSHSMEECEALCTRLAIMVKGAFRCMGTIQHLKSKFGDGYIVTMKIKSPKDDLLPDLNPVEQFFQGNFPGSVQRERHYNMLQFQVSSSSLARIFQLLLSHKDSLLIEEYSVTQTTLDQVFVNFAKQQTESHDLPLHPRAAGASRQAQDX

SEQ ID NO: 2 - protein, 1347 aa, synthetic construct
MGFVRQIQLLLWKNWTLRKRQKIRFVVELVWPLSLFLVLIWLRNANPLYSHHECHFPNKAMPSAGMLPWLQGIFCNVNNPCFQSPTPGESPGIVSNYNNSILARVYRDFQELLMNAPESQHLGRIWTELHILSQFMDTLRTHPERIAGRGIRIRDILKDEETLTLFLIKNIGLSDSVVYLLINSQVRPEQFAHGVPDLALKDIACSEALLERFIIFSQRRGAKTVRYALCSLSQGTLQWIEDTLYANVDFFKLFRVLPTLLDSRSQGINLRSWGGILSDMSPRIQEFIHRPSMQDLLWVTRPLMQNGGPETFTKLMGILSDLLCGYPEGGGSRVLSFNWYEDNNYKAFLGIDSTRKDPIYSYDRRTTSFCNALIQSLESNPLTKIAWRAAKPLLMGKILYTPDSPAARRILKNANSTFEELEHVRKLVKAWEEVGPQIWYFFDNSTQMNMIRDTLGNPTVKDFLNRQLGEEGITAEAILNFLYKGPRESQADDMANFDWRDIFNITDRTLRLVNQYLECLVLDKFESYNDETQLTQRALSLLEENMFWAGVVFPDMYPWTSSLPPHVKYKIRMDIDVVEKTNKIKDRYWDSGPRADPVEDFRYIWGGFAYLQDMVEQGITRSQVQAEAPVGIYLQQMPYPCFVDDSFMIILNRCFPIFMVLAWIYSVSMTVKSIVLEKELRLKETLKNQGVSNAVIWCTWFLDSFSIMSMSIFLLTIFIMHGRILHYSDPFILFLFLLAFSTATIMLCFLLSTFFSKASLAAACSGVIYFTLYLPHILCFAWQDRMTAELKKAVSLLSPVAFGFGTEYLVRFEEQGLGLQWSNIGNSPTEGDEFSFLLSMQMMLLDAAVYGLLAWYLDQVFPGDYGTPLPWYFLLQESYWLGGEGCSTREERALEKTEPLTEETEDPEHPEGIHDSFFEREHPGWVPGVCVKNLVKIFEPCGRPAVDRLNITFYENQITAFLGHNGAGKTTTLSILTGLLPPTSGTVLVGGRDIETSLDAVRQSLGMCPQHNILFHHLTVAEHMLFYAQLKGKSQEEAQLEMEAMLEDTGLHHKRNEEAQDLSGGMQRKLSVAIAFVGDAKVVILDEPTSGVDPYSRRSIWDLLLKYRSGRTIIMSTHHMDEADLLGDRIAIIAQGRLYCSGTPLFLKNCFGTGLYLTLVRKMKNIQSQRKGSEGTCSCSSKGFSTTCPAHVDDLTPEQVLDGDVNELMDVVLHHVPEAKLVECIGQELIFLLPNKNFKHRAYASLFRELEETLADLGLSSFGISDTPLEEIFLKVTEDSDSGPLFAGGAQQKRENVNPRHPCLGPREKAGQTPQDSNVCSPGAPAAHPEGQPPPEPECPGPQLNTG

SEQ ID NO: 3 - protein, 926 aa, synthetic construct
TQLVLQHVQALLVKRFQHTIRSHKDFLAQIVLPATFVFLALMLSIVIPPFGEYPALTLHPWIYGQQYTFFSMDEPGSEQFTVLADVLLNKPGFGNRCLKEGWLPEYPCGNSTPWKTPSVSPNITQLFQKQKWTQVNPSPSCRCSTREKLTMLPECPEGAGGLPPPQRTQRSTEILQDLTDRNISDFLVKTYPALIRSSLKSKFWVNEQRYGGISIGGKLPVVPITGEALVGFLSDLGRIMNVSGGPITREASKEIPDFLKHLETEDNIKVWFNNKGWHALVSFLNVAHNAILRASLPKDRSPEEYGITVISQPLNLTKEQLSEITVLTTSVDAVVAICVIFSMSFVPASFVLYLIQERVNKSKHLQFISGVSPTTYWVTNFLWDIMNYSVSAGLVVGIFIGFQKKAYTSPENLPALVALLLLYGWAVIPMMYPASFLFDVPSTAYVALSCANLFIGINSSAITFILELFENNRTLLRFNAVLRKLLIVFPHFCLGRGLIDLALSQAVTDVYARFGEEHSANPFHWDLIGKNLFAMVVEGVVYFLLTLLVQRHFFLSQWIAEPTKEPIVDEDDDVAEERQRIITGGNKTDILRLHELTKIYPGTSSPAVDRLCVGVRPGECFGLLGVNGAGKTTTFKMLTGDTTVTSGDATVAGKSILTNISEVHQNMGYCPQFDAIDELLTGREHLYLYARLRGVPAEEIEKVANWSIKSLGLTVYADCLAGTYSGGNKRKLSTAIALIGCPPLVLLDEPTTGMDPQARRMLWNVIVSIIREGRAVVLTSHSMEECEALCTRLAIMVKGAFRCMGTIQHLKSKFGDGYIVTMKIKSPKDDLLPDLNPVEQFFQGNFPGSVQRERHYNMLQFQVSSSSLARIFQLLLSHKDSLLIEEYSVTQTTLDQVFVNFAKQQTESHDLPLHPRAAGASRQAQD

SEQ ID NO: 4 - protein, 1152 aa, synthetic construct
MGFVRQIQLLLWKNWTLRKRQKIRFVVELVWPLSLFLVLIWLRNANPLYSHHECHFPNKAMPSAGMLPWLQGIFCNVNNPCFQSPTPGESPGIVSNYNNSILARVYRDFQELLMNAPESQHLGRIWTELHILSQFMDTLRTHPERIAGRGIRIRDILKDEETLTLFLIKNIGLSDSVVYLLINSQVRPEQFAHGVPDLALKDIACSEALLERFIIFSQRRGAKTVRYALCSLSQGTLQWIEDTLYANVDFFKLFRVLPTLLDSRSQGINLRSWGGILSDMSPRIQEFIHRPSMQDLLWVTRPLMQNGGPETFTKLMGILSDLLCGYPEGGGSRVLSFNWYEDNNYKAFLGIDSTRKDPIYSYDRRTTSFCNALIQSLESNPLTKIAWRAAKPLLMGKILYTPDSPAARRILKNANSTFEELEHVRKLVKAWEEVGPQIWYFFDNSTQMNMIRDTLGNPTVKDFLNRQLGEEGITAEAILNFLYKGPRESQADDMANFDWRDIFNITDRTLRLVNQYLECLVLDKFESYNDETQLTQRALSLLEENMFWAGVVFPDMYPWTSSLPPHVKYKIRMDIDVVEKTNKIKDRYWDSGPRADPVEDFRYIWGGFAYLQDMVEQGITRSQVQAEAPVGIYLQQMPYPCFVDDSFMIILNRCFPIFMVLAWIYSVSMTVKSIVLEKELRLKETLKNQGVSNAVIWCTWFLDSFSIMSMSIFLLTIFIMHGRILHYSDPFILFLFLLAFSTATIMLCFLLSTFFSKASLAAACSGVIYFTLYLPHILCFAWQDRMTAELKKAVSLLSPVAFGFGTEYLVRFEEQGLGLQWSNIGNSPTEGDEFSFLLSMQMMLLDAAVYGLLAWYLDQVFPGDYGTPLPWYFLLQESYWLGGEGCSTREERALEKTEPLTEETEDPEHPEGIHDSFFEREHPGWVPGVCVKNLVKIFEPCGRPAVDRLNITFYENQITAFLGHNGAGKTTTLSILTGLLPPTSGTVLVGGRDIETSLDAVRQSLGMCPQHNILFHHLTVAEHMLFYAQLKGKSQEEAQLEMEAMLEDTGLHHKRNEEAQDLSGGMQRKLSVAIAFVGDAKVVILDEPTSGVDPYSRRSIWDLLLKYRSGRTIIMSTHHMDEADLLGDRIAIIAQGRLYCSGTPLFLKNCFG

SEQ ID NO: 5 - protein, 816 aa, synthetic construct
TQLVLQHVQALLVKRFQHTIRSHKDFLAQIVLPATFVFLALMLSIVIPPFGEYPALTLHPWIYGQQYTFFSMDEPGSEQFTVLADVLLNKPGFGNRCLKEGWLPEYPCGNSTPWKTPSVSPNITQLFQKQKWTQVNPSPSCRCSTREKLTMLPECPEGAGGLPPPQRTQRSTEILQDLTDRNISDFLVKTYPALIRSSLKSKFWVNEQRYGGISIGGKLPVVPITGEALVGFLSDLGRIMNVSGGPITREASKEIPDFLKHLETEDNIKVWFNNKGWHALVSFLNVAHNAILRASLPKDRSPEEYGITVISQPLNLTKEQLSEITVLTTSVDAVVAICVIFSMSFVPASFVLYLIQERVNKSKHLQFISGVSPTTYWVTNFLWDIMNYSVSAGLVVGIFIGFQKKAYTSPENLPALVALLLLYGWAVIPMMYPASFLFDVPSTAYVALSCANLFIGINSSAITFILELFENNRTLLRFNAVLRKLLIVFPHFCLGRGLIDLALSQAVTDVYARFGEEHSANPFHWDLIGKNLFAMVVEGVVYFLLTLLVQRHFFLSQWIAEPTKEPIVDEDDDVAEERQRIITGGNKTDILRLHELTKIYPGTSSPAVDRLCVGVRPGECFGLLGVNGAGKTTTFKMLTGDTTVTSGDATVAGKSILTNISEVHQNMGYCPQFDAIDELLTGREHLYLYARLRGVPAEEIEKVANWSIKSLGLTVYADCLAGTYSGGNKRKLSTAIALIGCPPLVLLDEPTTGMDPQARRMLWNVIVSIIREGRAVVLTSHSMEECEALCTRLAIMVKGAFRCMGTIQHLKSKFGD

SEQ ID NO: 6 - protein, 227 aa, synthetic construct
DKTHTCPPCPAPELLGGPSVFLFPPKPKDTLMISRTPEVTCVVVDVSHEDPEVKFNWYVDGVEVHNAKTKPREEQYNSTYRVVSVLTVLHQDWLNGKEYKCKVSNKALPAPIEKTISKAKGQPREPQVYTLPPSREEMTKNQVSLWCLVKGFYPSDIAVEWESNGQPENNYKTTPPVLDSDGSFFLYSKLTVDKSRWQQGNVFSCSVMHEALHNHYTQKSLSLSPGK

SEQ ID NO: 7 - protein, 227 aa, synthetic construct
DKTHTCPPCPAPELLGGPSVFLFPPKPKDTLEASRTPEVTCVVVDVSHEDPEVKFNWYVDGVEVHNAKTKPREEQYNSTYRVVSVLTVLHQDWLNGKEYKCKVSNKALPAPIEKTISKAKGQPREPQVYTLPPSREEMTKNQVSLSCAVKGFYPSDIAVEWESNGQPENNYKTTPPVLDSDGSFFLVSKLTVDKSRWQQGNVFSCSVMHEALHNAYTQKSLSLSPGK

SEQ ID NO: 8 - protein, 1579 aa, synthetic construct
MGFVRQIQLLLWKNWTLRKRQKIRFVVELVWPLSLFLVLIWLRNANPLYSHHECHFPNKAMPSAGMLPWLQGIFCNVNNPCFQSPTPGESPGIVSNYNNSILARVYRDFQELLMNAPESQHLGRIWTELHILSQFMDTLRTHPERIAGRGIRIRDILKDEETLTLFLIKNIGLSDSVVYLLINSQVRPEQFAHGVPDLALKDIACSEALLERFIIFSQRRGAKTVRYALCSLSQGTLQWIEDTLYANVDFFKLFRVLPTLLDSRSQGINLRSWGGILSDMSPRIQEFIHRPSMQDLLWVTRPLMQNGGPETFTKLMGILSDLLCGYPEGGGSRVLSFNWYEDNNYKAFLGIDSTRKDPIYSYDRRTTSFCNALIQSLESNPLTKIAWRAAKPLLMGKILYTPDSPAARRILKNANSTFEELEHVRKLVKAWEEVGPQIWYFFDNSTQMNMIRDTLGNPTVKDFLNRQLGEEGITAEAILNFLYKGPRESQADDMANFDWRDIFNITDRTLRLVNQYLECLVLDKFESYNDETQLTQRALSLLEENMFWAGVVFPDMYPWTSSLPPHVKYKIRMDIDVVEKTNKIKDRYWDSGPRADPVEDFRYIWGGFAYLQDMVEQGITRSQVQAEAPVGIYLQQMPYPCFVDDSFMIILNRCFPIFMVLAWIYSVSMTVKSIVLEKELRLKETLKNQGVSNAVIWCTWFLDSFSIMSMSIFLLTIFIMHGRILHYSDPFILFLFLLAFSTATIMLCFLLSTFFSKASLAAACSGVIYFTLYLPHILCFAWQDRMTAELKKAVSLLSPVAFGFGTEYLVRFEEQGLGLQWSNIGNSPTEGDEFSFLLSMQMMLLDAAVYGLLAWYLDQVFPGDYGTPLPWYFLLQESYWLGGEGCSTREERALEKTEPLTEETEDPEHPEGIHDSFFEREHPGWVPGVCVKNLVKIFEPCGRPAVDRLNITFYENQITAFLGHNGAGKTTTLSILTGLLPPTSGTVLVGGRDIETSLDAVRQSLGMCPQHNILFHHLTVAEHMLFYAQLKGKSQEEAQLEMEAMLEDTGLHHKRNEEAQDLSGGMQRKLSVAIAFVGDAKVVILDEPTSGVDPYSRRSIWDLLLKYRSGRTIIMSTHHMDEADLLGDRIAIIAQGRLYCSGTPLFLKNCFGTGLYLTLVRKMKNIQSQRKGSEGTCSCSSKGFSTTCPAHVDDLTPEQVLDGDVNELMDVVLHHVPEAKLVECIGQELIFLLPNKNFKHRAYASLFRELEETLADLGLSSFGISDTPLEEIFLKVTEDSDSGPLFAGGAQQKRENVNPRHPCLGPREKAGQTPQDSNVCSPGAPAAHPEGQPPPEPECPGPQLNTGSGSGSDKTHTCPPCPAPELLGGPSVFLFPPKPKDTLMISRTPEVTCVVVDVSHEDPEVKFNWYVDGVEVHNAKTKPREEQYNSTYRVVSVLTVLHQDWLNGKEYKCKVSNKALPAPIEKTISKAKGQPREPQVYTLPPSREEMTKNQVSLWCLVKGFYPSDIAVEWESNGQPENNYKTTPPVLDSDGSFFLYSKLTVDKSRWQQGNVFSCSVMHEALHNHYTQKSLSLSPGK

SEQ ID NO: 9 - protein, 1579 aa, synthetic construct
MDKTHTCPPCPAPELLGGPSVFLFPPKPKDTLMISRTPEVTCVVVDVSHEDPEVKFNWYVDGVEVHNAKTKPREEQYNSTYRVVSVLTVLHQDWLNGKEYKCKVSNKALPAPIEKTISKAKGQPREPQVYTLPPSREEMTKNQVSLWCLVKGFYPSDIAVEWESNGQPENNYKTTPPVLDSDGSFFLYSKLTVDKSRWQQGNVFSCSVMHEALHNHYTQKSLSLSPGKSGSGSGFVRQIQLLLWKNWTLRKRQKIRFVVELVWPLSLFLVLIWLRNANPLYSHHECHFPNKAMPSAGMLPWLQGIFCNVNNPCFQSPTPGESPGIVSNYNNSILARVYRDFQELLMNAPESQHLGRIWTELHILSQFMDTLRTHPERIAGRGIRIRDILKDEETLTLFLIKNIGLSDSVVYLLINSQVRPEQFAHGVPDLALKDIACSEALLERFIIFSQRRGAKTVRYALCSLSQGTLQWIEDTLYANVDFFKLFRVLPTLLDSRSQGINLRSWGGILSDMSPRIQEFIHRPSMQDLLWVTRPLMQNGGPETFTKLMGILSDLLCGYPEGGGSRVLSFNWYEDNNYKAFLGIDSTRKDPIYSYDRRTTSFCNALIQSLESNPLTKIAWRAAKPLLMGKILYTPDSPAARRILKNANSTFEELEHVRKLVKAWEEVGPQIWYFFDNSTQMNMIRDTLGNPTVKDFLNRQLGEEGITAEAILNFLYKGPRESQADDMANFDWRDIFNITDRTLRLVNQYLECLVLDKFESYNDETQLTQRALSLLEENMFWAGVVFPDMYPWTSSLPPHVKYKIRMDIDVVEKTNKIKDRYWDSGPRADPVEDFRYIWGGFAYLQDMVEQGITRSQVQAEAPVGIYLQQMPYPCFVDDSFMIILNRCFPIFMVLAWIYSVSMTVKSIVLEKELRLKETLKNQGVSNAVIWCTWFLDSFSIMSMSIFLLTIFIMHGRILHYSDPFILFLFLLAFSTATIMLCFLLSTFFSKASLAAACSGVIYFTLYLPHILCFAWQDRMTAELKKAVSLLSPVAFGFGTEYLVRFEEQGLGLQWSNIGNSPTEGDEFSFLLSMQMMLLDAAVYGLLAWYLDQVFPGDYGTPLPWYFLLQESYWLGGEGCSTREERALEKTEPLTEETEDPEHPEGIHDSFFEREHPGWVPGVCVKNLVKIFEPCGRPAVDRLNITFYENQITAFLGHNGAGKTTTLSILTGLLPPTSGTVLVGGRDIETSLDAVRQSLGMCPQHNILFHHLTVAEHMLFYAQLKGKSQEEAQLEMEAMLEDTGLHHKRNEEAQDLSGGMQRKLSVAIAFVGDAKVVILDEPTSGVDPYSRRSIWDLLLKYRSGRTIIMSTHHMDEADLLGDRIAIIAQGRLYCSGTPLFLKNCFGTGLYLTLVRKMKNIQSQRKGSEGTCSCSSKGFSTTCPAHVDDLTPEQVLDGDVNELMDVVLHHVPEAKLVECIGQELIFLLPNKNFKHRAYASLFRELEETLADLGLSSFGISDTPLEEIFLKVTEDSDSGPLFAGGAQQKRENVNPRHPCLGPREKAGQTPQDSNVCSPGAPAAHPEGQPPPEPECPGPQLNTG

SEQ ID NO: 10 - protein, 1579 aa, synthetic construct
MDKTHTCPPCPAPELLGGPSVFLFPPKPKDTLEASRTPEVTCVVVDVSHEDPEVKFNWYVDGVEVHNAKTKPREEQYNSTYRVVSVLTVLHQDWLNGKEYKCKVSNKALPAPIEKTISKAKGQPREPQVYTLPPSREEMTKNQVSLSCAVKGFYPSDIAVEWESNGQPENNYKTTPPVLDSDGSFFLVSKLTVDKSRWQQGNVFSCSVMHEALHNAYTQKSLSLSPGKGSGSGGFVRQIQLLLWKNWTLRKRQKIRFVVELVWPLSLFLVLIWLRNANPLYSHHECHFPNKAMPSAGMLPWLQGIFCNVNNPCFQSPTPGESPGIVSNYNNSILARVYRDFQELLMNAPESQHLGRIWTELHILSQFMDTLRTHPERIAGRGIRIRDILKDEETLTLFLIKNIGLSDSVVYLLINSQVRPEQFAHGVPDLALKDIACSEALLERFIIFSQRRGAKTVRYALCSLSQGTLQWIEDTLYANVDFFKLFRVLPTLLDSRSQGINLRSWGGILSDMSPRIQEFIHRPSMQDLLWVTRPLMQNGGPETFTKLMGILSDLLCGYPEGGGSRVLSFNWYEDNNYKAFLGIDSTRKDPIYSYDRRTTSFCNALIQSLESNPLTKIAWRAAKPLLMGKILYTPDSPAARRILKNANSTFEELEHVRKLVKAWEEVGPQIWYFFDNSTQMNMIRDTLGNPTVKDFLNRQLGEEGITAEAILNFLYKGPRESQADDMANFDWRDIFNITDRTLRLVNQYLECLVLDKFESYNDETQLTQRALSLLEENMFWAGVVFPDMYPWTSSLPPHVKYKIRMDIDVVEKTNKIKDRYWDSGPRADPVEDFRYIWGGFAYLQDMVEQGITRSQVQAEAPVGIYLQQMPYPCFVDDSFMIILNRCFPIFMVLAWIYSVSMTVKSIVLEKELRLKETLKNQGVSNAVIWCTWFLDSFSIMSMSIFLLTIFIMHGRILHYSDPFILFLFLLAFSTATIMLCFLLSTFFSKASLAAACSGVIYFTLYLPHILCFAWQDRMTAELKKAVSLLSPVAFGFGTEYLVRFEEQGLGLQWSNIGNSPTEGDEFSFLLSMQMMLLDAAVYGLLAWYLDQVFPGDYGTPLPWYFLLQESYWLGGEGCSTREERALEKTEPLTEETEDPEHPEGIHDSFFEREHPGWVPGVCVKNLVKIFEPCGRPAVDRLNITFYENQITAFLGHNGAGKTTTLSILTGLLPPTSGTVLVGGRDIETSLDAVRQSLGMCPQHNILFHHLTVAEHMLFYAQLKGKSQEEAQLEMEAMLEDTGLHHKRNEEAQDLSGGMQRKLSVAIAFVGDAKVVILDEPTSGVDPYSRRSIWDLLLKYRSGRTIIMSTHHMDEADLLGDRIAIIAQGRLYCSGTPLFLKNCFGTGLYLTLVRKMKNIQSQRKGSEGTCSCSSKGFSTTCPAHVDDLTPEQVLDGDVNELMDVVLHHVPEAKLVECIGQELIFLLPNKNFKHRAYASLFRELEETLADLGLSSFGISDTPLEEIFLKVTEDSDSGPLFAGGAQQKRENVNPRHPCLGPREKAGQTPQDSNVCSPGAPAAHPEGQPPPEPECPGPQLNTG

SEQ ID NO: 11 - protein, 1159 aa, synthetic construct
MTQLVLQHVQALLVKRFQHTIRSHKDFLAQIVLPATFVFLALMLSIVIPPFGEYPALTLHPWIYGQQYTFFSMDEPGSEQFTVLADVLLNKPGFGNRCLKEGWLPEYPCGNSTPWKTPSVSPNITQLFQKQKWTQVNPSPSCRCSTREKLTMLPECPEGAGGLPPPQRTQRSTEILQDLTDRNISDFLVKTYPALIRSSLKSKFWVNEQRYGGISIGGKLPVVPITGEALVGFLSDLGRIMNVSGGPITREASKEIPDFLKHLETEDNIKVWFNNKGWHALVSFLNVAHNAILRASLPKDRSPEEYGITVISQPLNLTKEQLSEITVLTTSVDAVVAICVIFSMSFVPASFVLYLIQERVNKSKHLQFISGVSPTTYWVTNFLWDIMNYSVSAGLVVGIFIGFQKKAYTSPENLPALVALLLLYGWAVIPMMYPASFLFDVPSTAYVALSCANLFIGINSSAITFILELFENNRTLLRFNAVLRKLLIVFPHFCLGRGLIDLALSQAVTDVYARFGEEHSANPFHWDLIGKNLFAMVVEGVVYFLLTLLVQRHFFLSQWIAEPTKEPIVDEDDDVAEERQRIITGGNKTDILRLHELTKIYPGTSSPAVDRLCVGVRPGECFGLLGVNGAGKTTTFKMLTGDTTVTSGDATVAGKSILTNISEVHQNMGYCPQFDAIDELLTGREHLYLYARLRGVPAEEIEKVANWSIKSLGLTVYADCLAGTYSGGNKRKLSTAIALIGCPPLVLLDEPTTGMDPQARRMLWNVIVSIIREGRAVVLTSHSMEECEALCTRLAIMVKGAFRCMGTIQHLKSKFGDGYIVTMKIKSPKDDLLPDLNPVEQFFQGNFPGSVQRERHYNMLQFQVSSSSLARIFQLLLSHKDSLLIEEYSVTQTTLDQVFVNFAKQQTESHDLPLHPRAAGASRQAQDGSGSGDKTHTCPPCPAPELLGGPSVFLFPPKPKDTLMISRTPEVTCVVVDVSHEDPEVKFNWYVDGVEVHNAKTKPREEQYNSTYRVVSVLTVLHQDWLNGKEYKCKVSNKALPAPIEKTISKAKGQPREPQVYTLPPSREEMTKNQVSLWCLVKGFYPSDIAVEWESNGQPENNYKTTPPVLDSDGSFFLYSKLTVDKSRWQQGNVFSCSVMHEALHNHYTQKSLSLSPGK

SEQ ID NO: 12 - protein, 1159 aa, synthetic construct
MDKTHTCPPCPAPELLGGPSVFLFPPKPKDTLMISRTPEVTCVVVDVSHEDPEVKFNWYVDGVEVHNAKTKPREEQYNSTYRVVSVLTVLHQDWLNGKEYKCKVSNKALPAPIEKTISKAKGQPREPQVYTLPPSREEMTKNQVSLWCLVKGFYPSDIAVEWESNGQPENNYKTTPPVLDSDGSFFLYSKLTVDKSRWQQGNVFSCSVMHEALHNHYTQKSLSLSPGKGSGSGTQLVLQHVQALLVKRFQHTIRSHKDFLAQIVLPATFVFLALMLSIVIPPFGEYPALTLHPWIYGQQYTFFSMDEPGSEQFTVLADVLLNKPGFGNRCLKEGWLPEYPCGNSTPWKTPSVSPNITQLFQKQKWTQVNPSPSCRCSTREKLTMLPECPEGAGGLPPPQRTQRSTEILQDLTDRNISDFLVKTYPALIRSSLKSKFWVNEQRYGGISIGGKLPVVPITGEALVGFLSDLGRIMNVSGGPITREASKEIPDFLKHLETEDNIKVWFNNKGWHALVSFLNVAHNAILRASLPKDRSPEEYGITVISQPLNLTKEQLSEITVLTTSVDAVVAICVIFSMSFVPASFVLYLIQERVNKSKHLQFISGVSPTTYWVTNFLWDIMNYSVSAGLVVGIFIGFQKKAYTSPENLPALVALLLLYGWAVIPMMYPASFLFDVPSTAYVALSCANLFIGINSSAITFILELFENNRTLLRFNAVLRKLLIVFPHFCLGRGLIDLALSQAVTDVYARFGEEHSANPFHWDLIGKNLFAMVVEGVVYFLLTLLVQRHFFLSQWIAEPTKEPIVDEDDDVAEERQRIITGGNKTDILRLHELTKIYPGTSSPAVDRLCVGVRPGECFGLLGVNGAGKTTTFKMLTGDTTVTSGDATVAGKSILTNISEVHQNMGYCPQFDAIDELLTGREHLYLYARLRGVPAEEIEKVANWSIKSLGLTVYADCLAGTYSGGNKRKLSTAIALIGCPPLVLLDEPTTGMDPQARRMLWNVIVSIIREGRAVVLTSHSMEECEALCTRLAIMVKGAFRCMGTIQHLKSKFGDGYIVTMKIKSPKDDLLPDLNPVEQFFQGNFPGSVQRERHYNMLQFQVSSSSLARIFQLLLSHKDSLLIEEYSVTQTTLDQVFVNFAKQQTESHDLPLHPRAAGASRQAQD

SEQ ID NO: 13 - protein, 1160 aa, synthetic construct
MTQLVLQHVQALLVKRFQHTIRSHKDFLAQIVLPATFVFLALMLSIVIPPFGEYPALTLHPWIYGQQYTFFSMDEPGSEQFTVLADVLLNKPGFGNRCLKEGWLPEYPCGNSTPWKTPSVSPNITQLFQKQKWTQVNPSPSCRCSTREKLTMLPECPEGAGGLPPPQRTQRSTEILQDLTDRNISDFLVKTYPALIRSSLKSKFWVNEQRYGGISIGGKLPVVPITGEALVGFLSDLGRIMNVSGGPITREASKEIPDFLKHLETEDNIKVWFNNKGWHALVSFLNVAHNAILRASLPKDRSPEEYGITVISQPLNLTKEQLSEITVLTTSVDAVVAICVIFSMSFVPASFVLYLIQERVNKSKHLQFISGVSPTTYWVTNFLWDIMNYSVSAGLVVGIFIGFQKKAYTSPENLPALVALLLLYGWAVIPMMYPASFLFDVPSTAYVALSCANLFIGINSSAITFILELFENNRTLLRFNAVLRKLLIVFPHFCLGRGLIDLALSQAVTDVYARFGEEHSANPFHWDLIGKNLFAMVVEGVVYFLLTLLVQRHFFLSQWIAEPTKEPIVDEDDDVAEERQRIITGGNKTDILRLHELTKIYPGTSSPAVDRLCVGVRPGECFGLLGVNGAGKTTTFKMLTGDTTVTSGDATVAGKSILTNISEVHQNMGYCPQFDAIDELLTGREHLYLYARLRGVPAEEIEKVANWSIKSLGLTVYADCLAGTYSGGNKRKLSTAIALIGCPPLVLLDEPTTGMDPQARRMLWNVIVSIIREGRAVVLTSHSMEECEALCTRLAIMVKGAFRCMGTIQHLKSKFGDGYIVTMKIKSPKDDLLPDLNPVEQFFQGNFPGSVQRERHYNMLQFQVSSSSLARIFQLLLSHKDSLLIEEYSVTQTTLDQVFVNFAKQQTESHDLPLHPRAAGASRQAQDSGSGSDKTHTCPPCPAPELLGGPSVFLFPPKPKDTLEASRTPEVTCVVVDVSHEDPEVKFNWYVDGVEVHNAKTKPREEQYNSTYRVVSVLTVLHQDWLNGKEYKCKVSNKALPAPIEKTISKAKGQPREPQVYTLPPSREEMTKNQVSLSCAVKGFYPSDIAVEWESNGQPENNYKTTPPVLDSDGSFFLVSKLTVDKSRWQQGNVFSCSVMHEALHNAYTQKSLSLSPGKX

SEQ ID NO: 14 - protein, 1160 aa, synthetic construct
MDKTHTCPPCPAPELLGGPSVFLFPPKPKDTLEASRTPEVTCVVVDVSHEDPEVKFNWYVDGVEVHNAKTKPREEQYNSTYRVVSVLTVLHQDWLNGKEYKCKVSNKALPAPIEKTISKAKGQPREPQVYTLPPSREEMTKNQVSLSCAVKGFYPSDIAVEWESNGQPENNYKTTPPVLDSDGSFFLVSKLTVDKSRWQQGNVFSCSVMHEALHNAYTQKSLSLSPGKSGSGSTQLVLQHVQALLVKRFQHTIRSHKDFLAQIVLPATFVFLALMLSIVIPPFGEYPALTLHPWIYGQQYTFFSMDEPGSEQFTVLADVLLNKPGFGNRCLKEGWLPEYPCGNSTPWKTPSVSPNITQLFQKQKWTQVNPSPSCRCSTREKLTMLPECPEGAGGLPPPQRTQRSTEILQDLTDRNISDFLVKTYPALIRSSLKSKFWVNEQRYGGISIGGKLPVVPITGEALVGFLSDLGRIMNVSGGPITREASKEIPDFLKHLETEDNIKVWFNNKGWHALVSFLNVAHNAILRASLPKDRSPEEYGITVISQPLNLTKEQLSEITVLTTSVDAVVAICVIFSMSFVPASFVLYLIQERVNKSKHLQFISGVSPTTYWVTNFLWDIMNYSVSAGLVVGIFIGFQKKAYTSPENLPALVALLLLYGWAVIPMMYPASFLFDVPSTAYVALSCANLFIGINSSAITFILELFENNRTLLRFNAVLRKLLIVFPHFCLGRGLIDLALSQAVTDVYARFGEEHSANPFHWDLIGKNLFAMVVEGVVYFLLTLLVQRHFFLSQWIAEPTKEPIVDEDDDVAEERQRIITGGNKTDILRLHELTKIYPGTSSPAVDRLCVGVRPGECFGLLGVNGAGKTTTFKMLTGDTTVTSGDATVAGKSILTNISEVHQNMGYCPQFDAIDELLTGREHLYLYARLRGVPAEEIEKVANWSIKSLGLTVYADCLAGTYSGGNKRKLSTAIALIGCPPLVLLDEPTTGMDPQARRMLWNVIVSIIREGRAVVLTSHSMEECEALCTRLAIMVKGAFRCMGTIQHLKSKFGDGYIVTMKIKSPKDDLLPDLNPVEQFFQGNFPGSVQRERHYNMLQFQVSSSSLARIFQLLLSHKDSLLIEEYSVTQTTLDQVFVNFAKQQTESHDLPLHPRAAGASRQAQDX

SEQ ID NO: 15 - protein, 1384 aa, synthetic construct
MGFVRQIQLLLWKNWTLRKRQKIRFVVELVWPLSLFLVLIWLRNANPLYSHHECHFPNKAMPSAGMLPWLQGIFCNVNNPCFQSPTPGESPGIVSNYNNSILARVYRDFQELLMNAPESQHLGRIWTELHILSQFMDTLRTHPERIAGRGIRIRDILKDEETLTLFLIKNIGLSDSVVYLLINSQVRPEQFAHGVPDLALKDIACSEALLERFIIFSQRRGAKTVRYALCSLSQGTLQWIEDTLYANVDFFKLFRVLPTLLDSRSQGINLRSWGGILSDMSPRIQEFIHRPSMQDLLWVTRPLMQNGGPETFTKLMGILSDLLCGYPEGGGSRVLSFNWYEDNNYKAFLGIDSTRKDPIYSYDRRTTSFCNALIQSLESNPLTKIAWRAAKPLLMGKILYTPDSPAARRILKNANSTFEELEHVRKLVKAWEEVGPQIWYFFDNSTQMNMIRDTLGNPTVKDFLNRQLGEEGITAEAILNFLYKGPRESQADDMANFDWRDIFNITDRTLRLVNQYLECLVLDKFESYNDETQLTQRALSLLEENMFWAGVVFPDMYPWTSSLPPHVKYKIRMDIDVVEKTNKIKDRYWDSGPRADPVEDFRYIWGGFAYLQDMVEQGITRSQVQAEAPVGIYLQQMPYPCFVDDSFMIILNRCFPIFMVLAWIYSVSMTVKSIVLEKELRLKETLKNQGVSNAVIWCTWFLDSFSIMSMSIFLLTIFIMHGRILHYSDPFILFLFLLAFSTATIMLCFLLSTFFSKASLAAACSGVIYFTLYLPHILCFAWQDRMTAELKKAVSLLSPVAFGFGTEYLVRFEEQGLGLQWSNIGNSPTEGDEFSFLLSMQMMLLDAAVYGLLAWYLDQVFPGDYGTPLPWYFLLQESYWLGGEGCSTREERALEKTEPLTEETEDPEHPEGIHDSFFEREHPGWVPGVCVKNLVKIFEPCGRPAVDRLNITFYENQITAFLGHNGAGKTTTLSILTGLLPPTSGTVLVGGRDIETSLDAVRQSLGMCPQHNILFHHLTVAEHMLFYAQLKGKSQEEAQLEMEAMLEDTGLHHKRNEEAQDLSGGMQRKLSVAIAFVGDAKVVILDEPTSGVDPYSRRSIWDLLLKYRSGRTIIMSTHHMDEADLLGDRIAIIAQGRLYCSGTPLFLKNCFGGSGSGDKTHTCPPCPAPELLGGPSVFLFPPKPKDTLMISRTPEVTCVVVDVSHEDPEVKFNWYVDGVEVHNAKTKPREEQYNSTYRVVSVLTVLHQDWLNGKEYKCKVSNKALPAPIEKTISKAKGQPREPQVYTLPPSREEMTKNQVSLWCLVKGFYPSDIAVEWESNGQPENNYKTTPPVLDSDGSFFLYSKLTVDKSRWQQGNVFSCSVMHEALHNHYTQKSLSLSPGK

SEQ ID NO: 16 - protein, 1384 aa, synthetic construct
MDKTHTCPPCPAPELLGGPSVFLFPPKPKDTLMISRTPEVTCVVVDVSHEDPEVKFNWYVDGVEVHNAKTKPREEQYNSTYRVVSVLTVLHQDWLNGKEYKCKVSNKALPAPIEKTISKAKGQPREPQVYTLPPSREEMTKNQVSLWCLVKGFYPSDIAVEWESNGQPENNYKTTPPVLDSDGSFFLYSKLTVDKSRWQQGNVFSCSVMHEALHNHYTQKSLSLSPGKGSGSGGFVRQIQLLLWKNWTLRKRQKIRFVVELVWPLSLFLVLIWLRNANPLYSHHECHFPNKAMPSAGMLPWLQGIFCNVNNPCFQSPTPGESPGIVSNYNNSILARVYRDFQELLMNAPESQHLGRIWTELHILSQFMDTLRTHPERIAGRGIRIRDILKDEETLTLFLIKNIGLSDSVVYLLINSQVRPEQFAHGVPDLALKDIACSEALLERFIIFSQRRGAKTVRYALCSLSQGTLQWIEDTLYANVDFFKLFRVLPTLLDSRSQGINLRSWGGILSDMSPRIQEFIHRPSMQDLLWVTRPLMQNGGPETFTKLMGILSDLLCGYPEGGGSRVLSFNWYEDNNYKAFLGIDSTRKDPIYSYDRRTTSFCNALIQSLESNPLTKIAWRAAKPLLMGKILYTPDSPAARRILKNANSTFEELEHVRKLVKAWEEVGPQIWYFFDNSTQMNMIRDTLGNPTVKDFLNRQLGEEGITAEAILNFLYKGPRESQADDMANFDWRDIFNITDRTLRLVNQYLECLVLDKFESYNDETQLTQRALSLLEENMFWAGVVFPDMYPWTSSLPPHVKYKIRMDIDVVEKTNKIKDRYWDSGPRADPVEDFRYIWGGFAYLQDMVEQGITRSQVQAEAPVGIYLQQMPYPCFVDDSFMIILNRCFPIFMVLAWIYSVSMTVKSIVLEKELRLKETLKNQGVSNAVIWCTWFLDSFSIMSMSIFLLTIFIMHGRILHYSDPFILFLFLLAFSTATIMLCFLLSTFFSKASLAAACSGVIYFTLYLPHILCFAWQDRMTAELKKAVSLLSPVAFGFGTEYLVRFEEQGLGLQWSNIGNSPTEGDEFSFLLSMQMMLLDAAVYGLLAWYLDQVFPGDYGTPLPWYFLLQESYWLGGEGCSTREERALEKTEPLTEETEDPEHPEGIHDSFFEREHPGWVPGVCVKNLVKIFEPCGRPAVDRLNITFYENQITAFLGHNGAGKTTTLSILTGLLPPTSGTVLVGGRDIETSLDAVRQSLGMCPQHNILFHHLTVAEHMLFYAQLKGKSQEEAQLEMEAMLEDTGLHHKRNEEAQDLSGGMQRKLSVAIAFVGDAKVVILDEPTSGVDPYSRRSIWDLLLKYRSGRTIIMSTHHMDEADLLGDRIAIIAQGRLYCSGTPLFLKNCFG

SEQ ID NO: 17 - protein, 1384 aa, synthetic construct
MGFVRQIQLLLWKNWTLRKRQKIRFVVELVWPLSLFLVLIWLRNANPLYSHHECHFPNKAMPSAGMLPWLQGIFCNVNNPCFQSPTPGESPGIVSNYNNSILARVYRDFQELLMNAPESQHLGRIWTELHILSQFMDTLRTHPERIAGRGIRIRDILKDEETLTLFLIKNIGLSDSVVYLLINSQVRPEQFAHGVPDLALKDIACSEALLERFIIFSQRRGAKTVRYALCSLSQGTLQWIEDTLYANVDFFKLFRVLPTLLDSRSQGINLRSWGGILSDMSPRIQEFIHRPSMQDLLWVTRPLMQNGGPETFTKLMGILSDLLCGYPEGGGSRVLSFNWYEDNNYKAFLGIDSTRKDPIYSYDRRTTSFCNALIQSLESNPLTKIAWRAAKPLLMGKILYTPDSPAARRILKNANSTFEELEHVRKLVKAWEEVGPQIWYFFDNSTQMNMIRDTLGNPTVKDFLNRQLGEEGITAEAILNFLYKGPRESQADDMANFDWRDIFNITDRTLRLVNQYLECLVLDKFESYNDETQLTQRALSLLEENMFWAGVVFPDMYPWTSSLPPHVKYKIRMDIDVVEKTNKIKDRYWDSGPRADPVEDFRYIWGGFAYLQDMVEQGITRSQVQAEAPVGIYLQQMPYPCFVDDSFMIILNRCFPIFMVLAWIYSVSMTVKSIVLEKELRLKETLKNQGVSNAVIWCTWFLDSFSIMSMSIFLLTIFIMHGRILHYSDPFILFLFLLAFSTATIMLCFLLSTFFSKASLAAACSGVIYFTLYLPHILCFAWQDRMTAELKKAVSLLSPVAFGFGTEYLVRFEEQGLGLQWSNIGNSPTEGDEFSFLLSMQMMLLDAAVYGLLAWYLDQVFPGDYGTPLPWYFLLQESYWLGGEGCSTREERALEKTEPLTEETEDPEHPEGIHDSFFEREHPGWVPGVCVKNLVKIFEPCGRPAVDRLNITFYENQITAFLGHNGAGKTTTLSILTGLLPPTSGTVLVGGRDIETSLDAVRQSLGMCPQHNILFHHLTVAEHMLFYAQLKGKSQEEAQLEMEAMLEDTGLHHKRNEEAQDLSGGMQRKLSVAIAFVGDAKVVILDEPTSGVDPYSRRSIWDLLLKYRSGRTIIMSTHHMDEADLLGDRIAIIAQGRLYCSGTPLFLKNCFGGSGSGDKTHTCPPCPAPELLGGPSVFLFPPKPKDTLEASRTPEVTCVVVDVSHEDPEVKFNWYVDGVEVHNAKTKPREEQYNSTYRVVSVLTVLHQDWLNGKEYKCKVSNKALPAPIEKTISKAKGQPREPQVYTLPPSREEMTKNQVSLSCAVKGFYPSDIAVEWESNGQPENNYKTTPPVLDSDGSFFLVSKLTVDKSRWQQGNVFSCSVMHEALHNAYTQKSLSLSPGK

SEQ ID NO: 18 - protein, 1384 aa, synthetic construct
MDKTHTCPPCPAPELLGGPSVFLFPPKPKDTLEASRTPEVTCVVVDVSHEDPEVKFNWYVDGVEVHNAKTKPREEQYNSTYRVVSVLTVLHQDWLNGKEYKCKVSNKALPAPIEKTISKAKGQPREPQVYTLPPSREEMTKNQVSLSCAVKGFYPSDIAVEWESNGQPENNYKTTPPVLDSDGSFFLVSKLTVDKSRWQQGNVFSCSVMHEALHNAYTQKSLSLSPGKGSGSGGFVRQIQLLLWKNWTLRKRQKIRFVVELVWPLSLFLVLIWLRNANPLYSHHECHFPNKAMPSAGMLPWLQGIFCNVNNPCFQSPTPGESPGIVSNYNNSILARVYRDFQELLMNAPESQHLGRIWTELHILSQFMDTLRTHPERIAGRGIRIRDILKDEETLTLFLIKNIGLSDSVVYLLINSQVRPEQFAHGVPDLALKDIACSEALLERFIIFSQRRGAKTVRYALCSLSQGTLQWIEDTLYANVDFFKLFRVLPTLLDSRSQGINLRSWGGILSDMSPRIQEFIHRPSMQDLLWVTRPLMQNGGPETFTKLMGILSDLLCGYPEGGGSRVLSFNWYEDNNYKAFLGIDSTRKDPIYSYDRRTTSFCNALIQSLESNPLTKIAWRAAKPLLMGKILYTPDSPAARRILKNANSTFEELEHVRKLVKAWEEVGPQIWYFFDNSTQMNMIRDTLGNPTVKDFLNRQLGEEGITAEAILNFLYKGPRESQADDMANFDWRDIFNITDRTLRLVNQYLECLVLDKFESYNDETQLTQRALSLLEENMFWAGVVFPDMYPWTSSLPPHVKYKIRMDIDVVEKTNKIKDRYWDSGPRADPVEDFRYIWGGFAYLQDMVEQGITRSQVQAEAPVGIYLQQMPYPCFVDDSFMIILNRCFPIFMVLAWIYSVSMTVKSIVLEKELRLKETLKNQGVSNAVIWCTWFLDSFSIMSMSIFLLTIFIMHGRILHYSDPFILFLFLLAFSTATIMLCFLLSTFFSKASLAAACSGVIYFTLYLPHILCFAWQDRMTAELKKAVSLLSPVAFGFGTEYLVRFEEQGLGLQWSNIGNSPTEGDEFSFLLSMQMMLLDAAVYGLLAWYLDQVFPGDYGTPLPWYFLLQESYWLGGEGCSTREERALEKTEPLTEETEDPEHPEGIHDSFFEREHPGWVPGVCVKNLVKIFEPCGRPAVDRLNITFYENQITAFLGHNGAGKTTTLSILTGLLPPTSGTVLVGGRDIETSLDAVRQSLGMCPQHNILFHHLTVAEHMLFYAQLKGKSQEEAQLEMEAMLEDTGLHHKRNEEAQDLSGGMQRKLSVAIAFVGDAKVVILDEPTSGVDPYSRRSIWDLLLKYRSGRTIIMSTHHMDEADLLGDRIAIIAQGRLYCSGTPLFLKNCFG

SEQ ID NO: 19 - protein, 1049 aa, synthetic construct
MTQLVLQHVQALLVKRFQHTIRSHKDFLAQIVLPATFVFLALMLSIVIPPFGEYPALTLHPWIYGQQYTFFSMDEPGSEQFTVLADVLLNKPGFGNRCLKEGWLPEYPCGNSTPWKTPSVSPNITQLFQKQKWTQVNPSPSCRCSTREKLTMLPECPEGAGGLPPPQRTQRSTEILQDLTDRNISDFLVKTYPALIRSSLKSKFWVNEQRYGGISIGGKLPVVPITGEALVGFLSDLGRIMNVSGGPITREASKEIPDFLKHLETEDNIKVWFNNKGWHALVSFLNVAHNAILRASLPKDRSPEEYGITVISQPLNLTKEQLSEITVLTTSVDAVVAICVIFSMSFVPASFVLYLIQERVNKSKHLQFISGVSPTTYWVTNFLWDIMNYSVSAGLVVGIFIGFQKKAYTSPENLPALVALLLLYGWAVIPMMYPASFLFDVPSTAYVALSCANLFIGINSSAITFILELFENNRTLLRFNAVLRKLLIVFPHFCLGRGLIDLALSQAVTDVYARFGEEHSANPFHWDLIGKNLFAMVVEGVVYFLLTLLVQRHFFLSQWIAEPTKEPIVDEDDDVAEERQRIITGGNKTDILRLHELTKIYPGTSSPAVDRLCVGVRPGECFGLLGVNGAGKTTTFKMLTGDTTVTSGDATVAGKSILTNISEVHQNMGYCPQFDAIDELLTGREHLYLYARLRGVPAEEIEKVANWSIKSLGLTVYADCLAGTYSGGNKRKLSTAIALIGCPPLVLLDEPTTGMDPQARRMLWNVIVSIIREGRAVVLTSHSMEECEALCTRLAIMVKGAFRCMGTIQHLKSKFGDGSGSGDKTHTCPPCPAPELLGGPSVFLFPPKPKDTLMISRTPEVTCVVVDVSHEDPEVKFNWYVDGVEVHNAKTKPREEQYNSTYRVVSVLTVLHQDWLNGKEYKCKVSNKALPAPIEKTISKAKGQPREPQVYTLPPSREEMTKNQVSLWCLVKGFYPSDIAVEWESNGQPENNYKTTPPVLDSDGSFFLYSKLTVDKSRWQQGNVFSCSVMHEALHNHYTQKSLSLSPGK

SEQ ID NO: 20 - protein, 1049 aa, synthetic construct
MDKTHTCPPCPAPELLGGPSVFLFPPKPKDTLMISRTPEVTCVVVDVSHEDPEVKFNWYVDGVEVHNAKTKPREEQYNSTYRVVSVLTVLHQDWLNGKEYKCKVSNKALPAPIEKTISKAKGQPREPQVYTLPPSREEMTKNQVSLWCLVKGFYPSDIAVEWESNGQPENNYKTTPPVLDSDGSFFLYSKLTVDKSRWQQGNVFSCSVMHEALHNHYTQKSLSLSPGKGSGSGTQLVLQHVQALLVKRFQHTIRSHKDFLAQIVLPATFVFLALMLSIVIPPFGEYPALTLHPWIYGQQYTFFSMDEPGSEQFTVLADVLLNKPGFGNRCLKEGWLPEYPCGNSTPWKTPSVSPNITQLFQKQKWTQVNPSPSCRCSTREKLTMLPECPEGAGGLPPPQRTQRSTEILQDLTDRNISDFLVKTYPALIRSSLKSKFWVNEQRYGGISIGGKLPVVPITGEALVGFLSDLGRIMNVSGGPITREASKEIPDFLKHLETEDNIKVWFNNKGWHALVSFLNVAHNAILRASLPKDRSPEEYGITVISQPLNLTKEQLSEITVLTTSVDAVVAICVIFSMSFVPASFVLYLIQERVNKSKHLQFISGVSPTTYWVTNFLWDIMNYSVSAGLVVGIFIGFQKKAYTSPENLPALVALLLLYGWAVIPMMYPASFLFDVPSTAYVALSCANLFIGINSSAITFILELFENNRTLLRFNAVLRKLLIVFPHFCLGRGLIDLALSQAVTDVYARFGEEHSANPFHWDLIGKNLFAMVVEGVVYFLLTLLVQRHFFLSQWIAEPTKEPIVDEDDDVAEERQRIITGGNKTDILRLHELTKIYPGTSSPAVDRLCVGVRPGECFGLLGVNGAGKTTTFKMLTGDTTVTSGDATVAGKSILTNISEVHQNMGYCPQFDAIDELLTGREHLYLYARLRGVPAEEIEKVANWSIKSLGLTVYADCLAGTYSGGNKRKLSTAIALIGCPPLVLLDEPTTGMDPQARRMLWNVIVSIIREGRAVVLTSHSMEECEALCTRLAIMVKGAFRCMGTIQHLKSKFGD

SEQ ID NO: 21 - protein, 1049 aa, synthetic construct
MTQLVLQHVQALLVKRFQHTIRSHKDFLAQIVLPATFVFLALMLSIVIPPFGEYPALTLHPWIYGQQYTFFSMDEPGSEQFTVLADVLLNKPGFGNRCLKEGWLPEYPCGNSTPWKTPSVSPNITQLFQKQKWTQVNPSPSCRCSTREKLTMLPECPEGAGGLPPPQRTQRSTEILQDLTDRNISDFLVKTYPALIRSSLKSKFWVNEQRYGGISIGGKLPVVPITGEALVGFLSDLGRIMNVSGGPITREASKEIPDFLKHLETEDNIKVWFNNKGWHALVSFLNVAHNAILRASLPKDRSPEEYGITVISQPLNLTKEQLSEITVLTTSVDAVVAICVIFSMSFVPASFVLYLIQERVNKSKHLQFISGVSPTTYWVTNFLWDIMNYSVSAGLVVGIFIGFQKKAYTSPENLPALVALLLLYGWAVIPMMYPASFLFDVPSTAYVALSCANLFIGINSSAITFILELFENNRTLLRFNAVLRKLLIVFPHFCLGRGLIDLALSQAVTDVYARFGEEHSANPFHWDLIGKNLFAMVVEGVVYFLLTLLVQRHFFLSQWIAEPTKEPIVDEDDDVAEERQRIITGGNKTDILRLHELTKIYPGTSSPAVDRLCVGVRPGECFGLLGVNGAGKTTTFKMLTGDTTVTSGDATVAGKSILTNISEVHQNMGYCPQFDAIDELLTGREHLYLYARLRGVPAEEIEKVANWSIKSLGLTVYADCLAGTYSGGNKRKLSTAIALIGCPPLVLLDEPTTGMDPQARRMLWNVIVSIIREGRAVVLTSHSMEECEALCTRLAIMVKGAFRCMGTIQHLKSKFGDGSGSGDKTHTCPPCPAPELLGGPSVFLFPPKPKDTLEASRTPEVTCVVVDVSHEDPEVKFNWYVDGVEVHNAKTKPREEQYNSTYRVVSVLTVLHQDWLNGKEYKCKVSNKALPAPIEKTISKAKGQPREPQVYTLPPSREEMTKNQVSLSCAVKGFYPSDIAVEWESNGQPENNYKTTPPVLDSDGSFFLVSKLTVDKSRWQQGNVFSCSVMHEALHNAYTQKSLSLSPGK

SEQ ID NO: 22 - protein, 1049 aa, synthetic construct
MDKTHTCPPCPAPELLGGPSVFLFPPKPKDTLEASRTPEVTCVVVDVSHEDPEVKFNWYVDGVEVHNAKTKPREEQYNSTYRVVSVLTVLHQDWLNGKEYKCKVSNKALPAPIEKTISKAKGQPREPQVYTLPPSREEMTKNQVSLSCAVKGFYPSDIAVEWESNGQPENNYKTTPPVLDSDGSFFLVSKLTVDKSRWQQGNVFSCSVMHEALHNAYTQKSLSLSPGKGSGSGTQLVLQHVQALLVKRFQHTIRSHKDFLAQIVLPATFVFLALMLSIVIPPFGEYPALTLHPWIYGQQYTFFSMDEPGSEQFTVLADVLLNKPGFGNRCLKEGWLPEYPCGNSTPWKTPSVSPNITQLFQKQKWTQVNPSPSCRCSTREKLTMLPECPEGAGGLPPPQRTQRSTEILQDLTDRNISDFLVKTYPALIRSSLKSKFWVNEQRYGGISIGGKLPVVPITGEALVGFLSDLGRIMNVSGGPITREASKEIPDFLKHLETEDNIKVWFNNKGWHALVSFLNVAHNAILRASLPKDRSPEEYGITVISQPLNLTKEQLSEITVLTTSVDAVVAICVIFSMSFVPASFVLYLIQERVNKSKHLQFISGVSPTTYWVTNFLWDIMNYSVSAGLVVGIFIGFQKKAYTSPENLPALVALLLLYGWAVIPMMYPASFLFDVPSTAYVALSCANLFIGINSSAITFILELFENNRTLLRFNAVLRKLLIVFPHFCLGRGLIDLALSQAVTDVYARFGEEHSANPFHWDLIGKNLFAMVVEGVVYFLLTLLVQRHFFLSQWIAEPTKEPIVDEDDDVAEERQRIITGGNKTDILRLHELTKIYPGTSSPAVDRLCVGVRPGECFGLLGVNGAGKTTTFKMLTGDTTVTSGDATVAGKSILTNISEVHQNMGYCPQFDAIDELLTGREHLYLYARLRGVPAEEIEKVANWSIKSLGLTVYADCLAGTYSGGNKRKLSTAIALIGCPPLVLLDEPTTGMDPQARRMLWNVIVSIIREGRAVVLTSHSMEECEALCTRLAIMVKGAFRCMGTIQHLKSKFGD

SEQ ID NO: 23 - DNA, 6822 bp, Homo sapiens
  source 1..6822: mol_type = genomic DNA
atgggcttcgtgagacagatacagcttttgctctggaagaactggaccctgcggaaaaggcaaaagattcgctttgtggtggaactcgtgtggcctttatctttatttctggtcttgatctggttaaggaatgccaacccactctacagccatcatgaatgccatttccccaacaaggcgatgccctcagcaggaatgctgccgtggctccaggggatcttctgcaatgtgaacaatccctgttttcaaagccccaccccaggagaatctcctggaattgtgtcaaactataacaactccatcttggcaagggtatatcgagattttcaagaactcctcatgaatgcaccagagagccagcaccttggccgtatttggacagagctacacatcttgtcccaattcatggacaccctccggactcacccggagagaattgcaggaagaggaatacgaataagggatatcttgaaagatgaagaaacactgacactatttctcattaaaaacatcggcctgtctgactcagtggtctaccttctgatcaactctcaagtccgtccagagcagttcgctcatggagtcccggacctggcgctgaaggacatcgcctgcagcgaggccctcctggagcgcttcatcatcttcagccagagacgcggggcaaagacggtgcgctatgccctgtgctccctctcccagggcaccctacagtggatagaagacactctgtatgccaacgtggacttcttcaagctcttccgtgtgcttcccacactcctagacagccgttctcaaggtatcaatctgagatcttggggaggaatattatctgatatgtcaccaagaattcaagagtttatccatcggccgagtatgcaggacttgctgtgggtgaccaggcccctcatgcagaatggtggtccagagacctttacaaagctgatgggcatcctgtctgacctcctgtgtggctaccccgagggaggtggctctcgggtgctctccttcaactggtatgaagacaataactataaggcctttctggggattgactccacaaggaaggatcctatctattcttatgacagaagaacaacatccttttgtaatgcattgatccagagcctggagtcaaatcctttaaccaaaatcgcttggagggcggcaaagcctttgctgatgggaaaaatcctgtacactcctgattcacctgcagcacgaaggatactgaagaatgccaactcaacttttgaagaactggaacacgttaggaagttggtcaaagcctgggaagaagtagggccccagatctggtacttctttgacaacagcacacagatgaacatgatcagagataccctggggaacccaacagtaaaagactttttgaataggcagcttggtgaagaaggtattactgctgaagccatcctaaacttcctctacaagggccctcgggaaagccaggctgacgacatggccaacttcgactggagggacatatttaacatcactgatcgcaccctccgcctggtcaatcaatacctggagtgcttggtcctggataagtttgaaagctacaatgatgaaactcagctcacccaacgtgccctctctctactggaggaaaacatgttctgggccggagtggtattccctgacatgtatccctggaccagctctctaccaccccacgtgaagtataagatccgaatggacatagacgtggtggagaaaaccaataagattaaagacaggtattgggattctggtcccagagctgatcccgtggaagatttccggtacatctggggcgggtttgcctatctgcaggacatggttgaacaggggatcacaaggagccaggtgcaggcggaggctccagttggaatctacctccagcagatgccctacccctgcttcgtggacgattctttcatgatcatcctgaaccgctgtttccctatcttcatggtgctggcatggatctactctgtctccatgactgtgaagagcatcgtcttggagaaggagttgcgactgaaggagaccttgaaaaatcagggtgtctccaatgcagtgatttggtgtacctggttcctggacagcttctccatcatgtcgatgagcatcttcctcctgacgatattcatcatgcatggaagaatcctacattacagcgacccattcatcctcttcctgttcttgttggctttctccactgccaccatcatgctgtgctttctgctcagcaccttcttctccaaggccagtctggcagcagcctgtagtggtgtcatctatttcaccctctacctgccacacatcctgtgcttcgcctggcaggaccgcatgaccgctgagctgaagaaggctgtgagcttactgtctccggtggcatttggatttggcactgagtacctggttcgctttgaagagcaaggcctggggctgcagtggagcaacatcgggaacagtcccacggaaggggacgaattcagcttcctgctgtccatgcagatgatgctccttgatgctgctgtctatggcttactcgcttggtaccttgatcaggtgtttccaggagactatggaaccccacttccttggtactttcttctacaagagtcgtattggcttggcggtgaagggtgttcaaccagagaagaaagagccctggaaaagaccgagcccctaacagaggaaacggaggatccagagcacccagaaggaatacacgactccttctttgaacgtgagcatccagggtgggttcctggggtatgcgtgaagaatctggtaaagatttttgagccctgtggccggccagctgtggaccgtctgaacatcaccttctacgagaaccagatcaccgcattcctgggccacaatggagctgggaaaaccaccaccttgtccatcctgacgggtctgttgccaccaacctctgggactgtgctcgttgggggaagggacattgaaaccagcctggatgcagtccggcagagccttggcatgtgtccacagcacaacatcctgttccaccacctcacggtggctgagcacatgctgttctatgcccagctgaaaggaaagtcccaggaggaggcccagctggagatggaagccatgttggaggacacaggcctccaccacaagcggaatgaagaggctcaggacctatcaggtggcatgcagagaaagctgtcggttgccattgcctttgtgggagatgccaaggtggtgattctggacgaacccacctctggggtggacccttactcgagacgctcaatctgggatctgctcctgaagtatcgctcaggcagaaccatcatcatgtccactcaccacatggacgaggccgacctccttggggaccgcattgccatcattgcccagggaaggctctactgctcaggcaccccactcttcctgaagaactgctttggcacaggcttgtacttaaccttggtgcgcaagatgaaaaacatccagagccaaaggaaaggcagtgaggggacctgcagctgctcgtctaagggtttctccaccacgtgtccagcccacgtcgatgacctaactccagaacaagtcctggatggggatgtaaatgagctgatggatgtagttctccaccatgttccagaggcaaagctggtggagtgcattggtcaagaacttatcttccttcttccaaataagaacttcaagcacagagcatatgccagccttttcagagagctggaggagacgctggctgaccttggtctcagcagttttggaatttctgacactcccctggaagagatttttctgaaggtcacggaggattctgattcaggacctctgtttgcgggtggcgctcagcagaaaagagaaaacgtcaacccccgacacccctgcttgggtcccagagagaaggctggacagacaccccaggactccaatgtctgctccccaggggcgccggctgctcacccagagggccagcctcccccagagccagagtgcccaggcccgcagctcaacacggggacacagctggtcctccagcatgtgcaggcgctgctggtcaagagattccaacacaccatccgcagccacaaggacttcctggcgcagatcgtgctcccggctacctttgtgtttttggctctgatgctttctattgttatccctccttttggcgaataccccgctttgacccttcacccctggatatatgggcagcagtacaccttcttcagcatggatgaaccaggcagtgagcagttcacggtacttgcagacgtcctcctgaataagccaggctttggcaaccgctgcctgaaggaagggtggcttccggagtacccctgtggcaactcaacaccctggaagactccttctgtgtccccaaacatcacccagctgttccagaagcagaaatggacacaggtcaacccttcaccatcctgcaggtgcagcaccagggagaagctcaccatgctgccagagtgccccgagggtgccgggggcctcccgcccccccagagaacacagcgcagcacggaaattctacaagacctgacggacaggaacatctccgacttcttggtaaaaacgtatcctgctcttataagaagcagcttaaagagcaaattctgggtcaatgaacagaggtatggaggaatttccattggaggaaagctcccagtcgtccccatcacgggggaagcacttgttgggtttttaagcgaccttggccggatcatgaatgtgagcgggggccctatcactagagaggcctctaaagaaatacctgatttccttaaacatctagaaactgaagacaacattaaggtgtggtttaataacaaaggctggcatgccctggtcagctttctcaatgtggcccacaacgccatcttacgggccagcctgcctaaggacaggagccccgaggagtatggaatcaccgtcattagccaacccctgaacctgaccaaggagcagctctcagagattacagtgctgaccacttcagtggatgctgtggttgccatctgcgtgattttctccatgtccttcgtcccagccagctttgtcctttatttgatccaggagcgggtgaacaaatccaagcacctccagtttatcagtggagtgagccccaccacctactgggtgaccaacttcctctgggacatcatgaattattccgtgagtgctgggctggtggtgggcatcttcatcgggtttcagaagaaagcctacacttctccagaaaaccttcctgcccttgtggcactgctcctgctgtatggatgggcggtcattcccatgatgtacccagcatccttcctgtttgatgtccccagcacagcctatgtggctttatcttgtgctaatctgttcatcggcatcaacagcagtgctattaccttcatcttggaattatttgagaataaccggacgctgctcaggttcaacgccgtgctgaggaagctgctcattgtcttcccccacttctgcctgggccggggcctcattgaccttgcactgagccaggctgtgacagatgtctatgcccggtttggtgaggagcactctgcaaatccgttccactgggacctgattgggaagaacctgtttgccatggtggtggaaggggtggtgtacttcctcctgaccctgctggtccagcgccacttcttcctctcccaatggattgccgagcccactaaggagcccattgttgatgaagatgatgatgtggctgaagaaagacaaagaattattactggtggaaataaaactgacatcttaaggctacatgaactaaccaagatttatccaggcacctccagcccagcagtggacaggctgtgtgtcggagttcgccctggagagtgctttggcctcctgggagtgaatggtgccggcaaaacaaccacattcaagatgctcactggggacaccacagtgacctcaggggatgccaccgtagcaggcaagagtattttaaccaatatttctgaagtccatcaaaatatgggctactgtcctcagtttgatgcaattgatgagctgctcacaggacgagaacatctttacctttatgcccggcttcgaggtgtaccagcagaagaaatcgaaaaggttgcaaactggagtattaagagcctgggcctgactgtctacgccgactgcctggctggcacgtacagtgggggcaacaagcggaaactctccacagccatcgcactcattggctgcccaccgctggtgctgctggatgagcccaccacagggatggacccccaggcacgccgcatgctgtggaacgtcatcgtgagcatcatcagagaagggagggctgtggtcctcacatcccacagcatggaagaatgtgaggcactgtgtacccggctggccatcatggtaaagggcgcctttcgatgtatgggcaccattcagcatctcaagtccaaatttggagatggctatatcgtcacaatgaagatcaaatccccgaaggacgacctgcttcctgacctgaaccctgtggagcagttcttccaggggaacttcccaggcagtgtgcagagggagaggcactacaacatgctccagttccaggtctcctcctcctccctggcgaggatcttccagctcctcctctcccacaaggacagcctgctcatcgaggagtactcagtcacacagaccacactggaccaggtgtttgtaaattttgctaaacagcagactgaaagtcatgacctccctctgcaccctcgagctgctggagccagtcgacaagcccaggactga

SEQ ID NO: 24 - DNA, 6822 bp, synthetic construct
  source 1..6822: mol_type = other DNA
atgggattcgtgcggcagatccagcttctgctctggaagaattggaccctgcgtaaacggcagaagattagatttgtggtggagctggtgtggcctctgagcctgttcttggtgctgatctggctgcgaaacgccaaccctctgtactcccaccatgagtgtcacttccctaacaaggccatgccttctgctggcatgctgccttggctgcagggcatcttctgcaacgtgaacaacccctgcttccagagccccacccctggagagtctcccggcatcgtcagtaactacaacaactccatcctcgccagagtgtacagagatttccaggagctgctgatgaacgcccctgagtctcaacacctggggagaatctggaccgagctccatatactgtcacagttcatggataccctacggacccaccccgaacggatcgccggcagaggcattagaatccgggatatccttaaggacgaagagacactgactctttttctgattaagaatatcggattgtctgattcggtggtgtacctgctgatcaacagccaggtgagacctgagcagttcgcccacggcgtgcctgacttagcgctgaaggacattgcctgctctgaggccttgctggaaagattcatcatcttctctcagcggcggggggccaagacagttcggtacgccctgtgcagcctgagccagggcaccttgcagtggatcgaagacaccctgtatgctaacgtggacttctttaaactgtttagagtgttgccaaccttactggacagccggagccagggcatcaacctgagatcctggggtggaatcctgagcgatatgagccccagaatccaggagttcatccaccggcctagcatgcaggacttgctgtgggtgactcgtcccctgatgcaaaacggaggaccagaaacatttacaaagcttatgggcatcctgagcgacctcttgtgcggctaccctgagggcggcggcagccgggtgttaagctttaactggtacgaggacaacaactacaaggccttccttggtatcgatagcacacgaaaggacccaatctacagctacgaccgtagaacaaccagtttctgcaacgccctgatccagtcccttgaatctaatcctttgacaaagatcgcttggcgggccgccaagcctctgctgatgggcaagatcctgtacacccctgacagccctgccgccagaagaatcctaaagaatgccaacagcactttcgaggaactcgaacacgtgcggaagctggtcaaagcctgggaggaggtgggccctcaaatctggtacttcttcgataactccacccagatgaacatgatcagagacaccttgggaaatccgaccgtgaaggacttcctgaatagacagctaggtgaggagggaatcaccgccgaggccatcctgaactttctgtacaaaggccctcgggagtcccaggctgatgacatggccaattttgactggagagacatattcaacatcacagaccgtacccttagactggtgaaccagtacctggaatgcttagtcctggataagttcgaaagctacaacgacgagacccagctgacccaacgggcactgtctctactggaggagaatatgttctgggccggtgtggtgttccctgacatgtacccctggacaagcagcctgccacctcacgtgaaatacaagatccggatggacattgacgtggtggaaaagacaaacaagatcaaggacagatactgggacagcggacctagggccgatcctgtggaggatttccggtacatctggggtggcttcgcttacctgcaggacatggtggaacagggcatcacgagaagccaggtgcaggctgaggcccctgtgggaatctacctccaacagatgccctacccctgcttcgtggacgacagcttcatgatcatcctgaatagatgtttcccaatcttcatggtgctggcctggatctacagcgtgtccatgactgtgaagtccatcgtgctggagaaggagctgcggctaaaagagactctgaagaatcagggcgtgagcaacgccgtaatctggtgcacctggttcctggactccttctccatcatgagcatgagcatcttcctactgacaatctttatcatgcacggcagaattctgcactacagcgaccctttcatcctgtttctttttttgctggctttcagcaccgccaccatcatgctgtgcttcctgttaagcaccttcttctcaaaggccagcctagctgcagcatgctccggcgtcatctactttactttatacctgccccacatcctgtgtttcgcctggcaggacagaatgacagccgagctgaaaaaggccgtatccctgttgagccccgtggccttcgggtttggaaccgagtacctggtacggttcgaggaacaaggcctgggcctgcagtggtccaacatcggcaactcgccgaccgagggcgacgaattcagcttcctgctgtccatgcagatgatgctgctggatgccgcagtgtatggcctcctggcttggtacttggaccaggtgttccccggcgactacgggactccactgccatggtactttctgctgcaggagagctactggctgggcggcgagggctgcagcaccagagaggaaagagccctggagaagacagagcctctgactgaagaaaccgaagaccctgagcaccctgaggggatacacgactcttttttcgagagggaacatcctggatgggtccctggcgtttgcgtgaagaacctggtgaagatcttcgagccttgtggcaggccagccgtggatagactgaatatcaccttctacgagaaccagatcaccgccttcctgggccacaacggcgcgggaaagaccacaactctgagcatcctgaccggactgctgcctccaacttccggcaccgtgctcgtcggcggcagggacatcgagaccagtctggacgccgtgagacagagcctcggcatgtgccctcagcacaatatcctgtttcaccacttaaccgttgcagaacacatgctgttctacgcccagttaaaaggcaagtcgcaggaggaggcccagctggagatggaagcaatgctcgaagatacaggcctgcaccataagagaaacgaagaggcccaggatctctccggcggcatgcagagaaaactgagcgtagccatcgccttcgtgggagatgcaaaggtggtaatcctagatgagcctacatctggggtggacccgtacagccggcgcagtatttgggatttactgctgaagtacagaagcggtagaaccatcatcatgtctacccaccacatggacgaggctgatctgctgggagatcggatcgccataatcgcccagggaagactgtattgcagcggcacaccactgttcctcaaaaactgctttgggacgggactgtacctgacgctggtccggaaaatgaagaacatccagtcccagagaaagggctctgaagggacctgttcttgcagctctaagggcttcagtaccacctgccctgcccacgtggacgacctgactcccgaacaggtgctggacggcgatgtgaacgagctgatggacgtggtgctgcatcacgtacccgaagccaagctggttgaatgcatcggccaggagctcattttccttcttcctaacaagaacttcaagcacagagcttatgcctctctgttcagggaactggaggaaaccctagccgacctgggtctgtctagcttcggcatctctgacacacctctggaggagatctttctgaaagtgactgaggattctgatagcggaccactgttcgccggaggcgctcagcagaagagagaaaacgtcaatcctagacacccttgtctgggaccgagagagaaggccggccagacccctcaagattccaatgtgtgtagccctggcgcccccgctgctcacccagagggccagcctcctcctgaacctgaatgccccggcccccagctgaacaccggcactcagctggtcctgcagcacgtgcaggccctgctggtgaagcgcttccagcacacaatccgcagtcataaagacttcctcgctcagatcgtgctcccggctacattcgtgtttctggccctcatgctgtctatcgtgatcccacctttcggcgaataccctgcgctgaccctgcacccctggatatacggtcagcaatacacctttttcagcatggacgagcccggaagcgagcagttcaccgtgctggccgatgtgctgctgaacaagcctggcttcggcaaccggtgcctgaaagaaggatggctgccagagtacccctgcggcaatagcacaccttggaagacccctagcgtgtcccctaacatcacccagctgtttcaaaaacagaaatggacccaagtgaatccttcaccttcatgcagatgttctacacgtgaaaagctgaccatgttacccgagtgtcctgaaggagctggcggccttcctcctccccagaggacccagagaagcaccgaaatcctgcaggacctgacagaccggaacatctccgactttcttgtcaagacctaccctgccctgattaggagtagcctgaaatctaagttttgggttaatgaacagcggtacggcggcatcagcatcggcggtaagctgcccgtggtgcctattacaggcgaggccctggtgggcttcctcagtgatttgggacggataatgaacgtgagtggcggcccaatcacacgggaagccagcaaagagatccctgatttcctgaagcacctggaaacagaggataatataaaggtgtggttcaacaacaaaggctggcacgccctggtgagtttcctcaacgtagcccacaacgctatcctgagagcctctctacctaaggacagaagccccgaagagtacggcattaccgtgatcagccagcccctaaacctgacaaaggaacagctgagcgagattaccgtcctgacaacctccgttgacgcggtggtggcgatctgcgtgatcttttctatgagcttcgtgcctgccagcttcgtgctgtacctgatccaggagagagtgaacaagagcaagcacctgcaatttatttctggcgtgagcccaaccacctactgggtgaccaacttcctgtgggacatcatgaactacagcgtgtctgccggcctggtggtaggcatcttcatcggcttccagaagaaggcctacacctctcctgagaatctgcctgctctcgtggccctgctgctgctgtacggctgggccgtgatccccatgatgtaccccgctagcttcttatttgacgtgccctcaacagcatacgtggccttatcctgcgccaacctgtttataggaatcaattctagcgccatcacgttcatcctagaactgttcgagaacaaccggacactgctgcgattcaacgccgtcctgcggaagctcctgattgtgttccctcatttctgtctgggcagagggctgatcgacctggccctgagccaagccgtgaccgatgtgtacgcgagattcggcgaggagcactccgccaaccctttccactgggacctgatcggcaagaatctgttcgccatggttgtggagggtgtggtgtacttcctgcttacactgctggtgcagagacacttcttcctgtcccagtggattgccgaacccaccaaggaacccatcgtcgacgaggatgacgacgtggccgaggagagacagagaatcatcaccggcgggaacaaaaccgacatcctgagactccacgagctgacaaagatctatcctggcacaagcagccccgccgtggatcggctgtgtgtgggcgtcagacctggcgagtgcttcggcctgctgggcgtgaacggcgccggcaagaccacaaccttcaagatgctgaccggcgacaccacggtgacctccggcgacgccacagtggccggcaaaagcatcctcacaaacatctccgaagtgcaccagaacatgggctactgcccccagtttgatgctatagacgagctgttgaccggtagagaacacctgtacctgtacgccagactgagaggcgtgcctgctgaagagatcgaaaaggtggcaaactggagcatcaagtcactgggcctgacagtctacgccgactgcctggccggcacgtactctggcggcaataagcggaaactgagcaccgccattgccttgattggatgtccgcctctggtgctgctggacgagccgacaacaggcatggacccccaagcccggagaatgctgtggaacgtgatcgtgagcataatcagagagggcagagccgtggttttgacttctcacagcatggaagaatgtgaagcgctctgcacccggcttgccatcatggtcaaaggcgccttccggtgcatgggcaccattcagcacctgaagtccaagttcggcgacggctacatcgtgacaatgaagatcaaatctcccaaggacgacctgcttccagatctgaaccctgtggaacagttcttccagggaaatttccctggaagcgtgcagagagagagacactacaatatgctgcagtttcaggtaagcagcagcagccttgctcggatctttcagctgctgcttagccacaaggactctctgctgatcgaagagtacagcgtgacccagacaacgcttgatcaggtgttcgtgaacttcgccaagcagcaaaccgagagccatgatctgcctcttcacccacgagctgccggcgccagcagacaggcccaggactga

SEQ ID NO: 25 - DNA, 4041 bp, synthetic construct
  source 1..4041: mol_type = other DNA
atgggattcgtgcggcagatccagcttctgctctggaagaattggaccctgcgtaaacggcagaagattagatttgtggtggagctggtgtggcctctgagcctgttcttggtgctgatctggctgcgaaacgccaaccctctgtactcccaccatgagtgtcacttccctaacaaggccatgccttctgctggcatgctgccttggctgcagggcatcttctgcaacgtgaacaacccctgcttccagagccccacccctggagagtctcccggcatcgtcagtaactacaacaactccatcctcgccagagtgtacagagatttccaggagctgctgatgaacgcccctgagtctcaacacctggggagaatctggaccgagctccatatactgtcacagttcatggataccctacggacccaccccgaacggatcgccggcagaggcattagaatccgggatatccttaaggacgaagagacactgactctttttctgattaagaatatcggattgtctgattcggtggtgtacctgctgatcaacagccaggtgagacctgagcagttcgcccacggcgtgcctgacttagcgctgaaggacattgcctgctctgaggccttgctggaaagattcatcatcttctctcagcggcggggggccaagacagttcggtacgccctgtgcagcctgagccagggcaccttgcagtggatcgaagacaccctgtatgctaacgtggacttctttaaactgtttagagtgttgccaaccttactggacagccggagccagggcatcaacctgagatcctggggtggaatcctgagcgatatgagccccagaatccaggagttcatccaccggcctagcatgcaggacttgctgtgggtgactcgtcccctgatgcaaaacggaggaccagaaacatttacaaagcttatgggcatcctgagcgacctcttgtgcggctaccctgagggcggcggcagccgggtgttaagctttaactggtacgaggacaacaactacaaggccttccttggtatcgatagcacacgaaaggacccaatctacagctacgaccgtagaacaaccagtttctgcaacgccctgatccagtcccttgaatctaatcctttgacaaagatcgcttggcgggccgccaagcctctgctgatgggcaagatcctgtacacccctgacagccctgccgccagaagaatcctaaagaatgccaacagcactttcgaggaactcgaacacgtgcggaagctggtcaaagcctgggaggaggtgggccctcaaatctggtacttcttcgataactccacccagatgaacatgatcagagacaccttgggaaatccgaccgtgaaggacttcctgaatagacagctaggtgaggagggaatcaccgccgaggccatcctgaactttctgtacaaaggccctcgggagtcccaggctgatgacatggccaattttgactggagagacatattcaacatcacagaccgtacccttagactggtgaaccagtacctggaatgcttagtcctggataagttcgaaagctacaacgacgagacccagctgacccaacgggcactgtctctactggaggagaatatgttctgggccggtgtggtgttccctgacatgtacccctggacaagcagcctgccacctcacgtgaaatacaagatccggatggacattgacgtggtggaaaagacaaacaagatcaaggacagatactgggacagcggacctagggccgatcctgtggaggatttccggtacatctggggtggcttcgcttacctgcaggacatggtggaacagggcatcacgagaagccaggtgcaggctgaggcccctgtgggaatctacctccaacagatgccctacccctgcttcgtggacgacagcttcatgatcatcctgaatagatgtttcccaatcttcatggtgctggcctggatctacagcgtgtccatgactgtgaagtccatcgtgctggagaaggagctgcggctaaaagagactctgaagaatcagggcgtgagcaacgccgtaatctggtgcacctggttcctggactccttctccatcatgagcatgagcatcttcctactgacaatctttatcatgcacggcagaattctgcactacagcgaccctttcatcctgtttctttttttgctggctttcagcaccgccaccatcatgctgtgcttcctgttaagcaccttcttctcaaaggccagcctagctgcagcatgctccggcgtcatctactttactttatacctgccccacatcctgtgtttcgcctggcaggacagaatgacagccgagctgaaaaaggccgtatccctgttgagccccgtggccttcgggtttggaaccgagtacctggtacggttcgaggaacaaggcctgggcctgcagtggtccaacatcggcaactcgccgaccgagggcgacgaattcagcttcctgctgtccatgcagatgatgctgctggatgccgcagtgtatggcctcctggcttggtacttggaccaggtgttccccggcgactacgggactccactgccatggtactttctgctgcaggagagctactggctgggcggcgagggctgcagcaccagagaggaaagagccctggagaagacagagcctctgactgaagaaaccgaagaccctgagcaccctgaggggatacacgactcttttttcgagagggaacatcctggatgggtccctggcgtttgcgtgaagaacctggtgaagatcttcgagccttgtggcaggccagccgtggatagactgaatatcaccttctacgagaaccagatcaccgccttcctgggccacaacggcgcgggaaagaccacaactctgagcatcctgaccggactgctgcctccaacttccggcaccgtgctcgtcggcggcagggacatcgagaccagtctggacgccgtgagacagagcctcggcatgtgccctcagcacaatatcctgtttcaccacttaaccgttgcagaacacatgctgttctacgcccagttaaaaggcaagtcgcaggaggaggcccagctggagatggaagcaatgctcgaagatacaggcctgcaccataagagaaacgaagaggcccaggatctctccggcggcatgcagagaaaactgagcgtagccatcgccttcgtgggagatgcaaaggtggtaatcctagatgagcctacatctggggtggacccgtacagccggcgcagtatttgggatttactgctgaagtacagaagcggtagaaccatcatcatgtctacccaccacatggacgaggctgatctgctgggagatcggatcgccataatcgcccagggaagactgtattgcagcggcacaccactgttcctcaaaaactgctttgggacgggactgtacctgacgctggtccggaaaatgaagaacatccagtcccagagaaagggctctgaagggacctgttcttgcagctctaagggcttcagtaccacctgccctgcccacgtggacgacctgactcccgaacaggtgctggacggcgatgtgaacgagctgatggacgtggtgctgcatcacgtacccgaagccaagctggttgaatgcatcggccaggagctcattttccttcttcctaacaagaacttcaagcacagagcttatgcctctctgttcagggaactggaggaaaccctagccgacctgggtctgtctagcttcggcatctctgacacacctctggaggagatctttctgaaagtgactgaggattctgatagcggaccactgttcgccggaggcgctcagcagaagagagaaaacgtcaatcctagacacccttgtctgggaccgagagagaaggccggccagacccctcaagattccaatgtgtgtagccctggcgcccccgctgctcacccagagggccagcctcctcctgaacctgaatgccccggcccccagctgaacaccggc

SEQ ID NO: 26 - DNA, 2778 bp, synthetic construct
  source 1..2778: mol_type = other DNA
actcagctggtcctgcagcacgtgcaggccctgctggtgaagcgcttccagcacacaatccgcagtcataaagacttcctcgctcagatcgtgctcccggctacattcgtgtttctggccctcatgctgtctatcgtgatcccacctttcggcgaataccctgcgctgaccctgcacccctggatatacggtcagcaatacacctttttcagcatggacgagcccggaagcgagcagttcaccgtgctggccgatgtgctgctgaacaagcctggcttcggcaaccggtgcctgaaagaaggatggctgccagagtacccctgcggcaatagcacaccttggaagacccctagcgtgtcccctaacatcacccagctgtttcaaaaacagaaatggacccaagtgaatccttcaccttcatgcagatgttctacacgtgaaaagctgaccatgttacccgagtgtcctgaaggagctggcggccttcctcctccccagaggacccagagaagcaccgaaatcctgcaggacctgacagaccggaacatctccgactttcttgtcaagacctaccctgccctgattaggagtagcctgaaatctaagttttgggttaatgaacagcggtacggcggcatcagcatcggcggtaagctgcccgtggtgcctattacaggcgaggccctggtgggcttcctcagtgatttgggacggataatgaacgtgagtggcggcccaatcacacgggaagccagcaaagagatccctgatttcctgaagcacctggaaacagaggataatataaaggtgtggttcaacaacaaaggctggcacgccctggtgagtttcctcaacgtagcccacaacgctatcctgagagcctctctacctaaggacagaagccccgaagagtacggcattaccgtgatcagccagcccctaaacctgacaaaggaacagctgagcgagattaccgtcctgacaacctccgttgacgcggtggtggcgatctgcgtgatcttttctatgagcttcgtgcctgccagcttcgtgctgtacctgatccaggagagagtgaacaagagcaagcacctgcaatttatttctggcgtgagcccaaccacctactgggtgaccaacttcctgtgggacatcatgaactacagcgtgtctgccggcctggtggtaggcatcttcatcggcttccagaagaaggcctacacctctcctgagaatctgcctgctctcgtggccctgctgctgctgtacggctgggccgtgatccccatgatgtaccccgctagcttcttatttgacgtgccctcaacagcatacgtggccttatcctgcgccaacctgtttataggaatcaattctagcgccatcacgttcatcctagaactgttcgagaacaaccggacactgctgcgattcaacgccgtcctgcggaagctcctgattgtgttccctcatttctgtctgggcagagggctgatcgacctggccctgagccaagccgtgaccgatgtgtacgcgagattcggcgaggagcactccgccaaccctttccactgggacctgatcggcaagaatctgttcgccatggttgtggagggtgtggtgtacttcctgcttacactgctggtgcagagacacttcttcctgtcccagtggattgccgaacccaccaaggaacccatcgtcgacgaggatgacgacgtggccgaggagagacagagaatcatcaccggcgggaacaaaaccgacatcctgagactccacgagctgacaaagatctatcctggcacaagcagccccgccgtggatcggctgtgtgtgggcgtcagacctggcgagtgcttcggcctgctgggcgtgaacggcgccggcaagaccacaaccttcaagatgctgaccggcgacaccacggtgacctccggcgacgccacagtggccggcaaaagcatcctcacaaacatctccgaagtgcaccagaacatgggctactgcccccagtttgatgctatagacgagctgttgaccggtagagaacacctgtacctgtacgccagactgagaggcgtgcctgctgaagagatcgaaaaggtggcaaactggagcatcaagtcactgggcctgacagtctacgccgactgcctggccggcacgtactctggcggcaataagcggaaactgagcaccgccattgccttgattggatgtccgcctctggtgctgctggacgagccgacaacaggcatggacccccaagcccggagaatgctgtggaacgtgatcgtgagcataatcagagagggcagagccgtggttttgacttctcacagcatggaagaatgtgaagcgctctgcacccggcttgccatcatggtcaaaggcgccttccggtgcatgggcaccattcagcacctgaagtccaagttcggcgacggctacatcgtgacaatgaagatcaaatctcccaaggacgacctgcttccagatctgaaccctgtggaacagttcttccagggaaatttccctggaagcgtgcagagagagagacactacaatatgctgcagtttcaggtaagcagcagcagccttgctcggatctttcagctgctgcttagccacaaggactctctgctgatcgaagagtacagcgtgacccagacaacgcttgatcaggtgttcgtgaacttcgccaagcagcaaaccgagagccatgatctgcctcttcacccacgagctgccggcgccagcagacaggcccaggac

SEQ ID NO: 27 - DNA, 3456 bp, synthetic construct
  source 1..3456: mol_type = other DNA
atgggcttcgtgagacagatacagcttttgctctggaagaactggaccctgcggaaaaggcaaaagattcgctttgtggtggaactcgtgtggcctttatctttatttctggtcttgatctggttaaggaatgccaacccactctacagccatcatgaatgccatttccccaacaaggcgatgccctcagcaggaatgctgccgtggctccaggggatcttctgcaatgtgaacaatccctgttttcaaagccccaccccaggagaatctcctggaattgtgtcaaactataacaactccatcttggcaagggtatatcgagattttcaagaactcctcatgaatgcaccagagagccagcaccttggccgtatttggacagagctacacatcttgtcccaattcatggacaccctccggactcacccggagagaattgcaggaagaggaatacgaataagggatatcttgaaagatgaagaaacactgacactatttctcattaaaaacatcggcctgtctgactcagtggtctaccttctgatcaactctcaagtccgtccagagcagttcgctcatggagtcccggacctggcgctgaaggacatcgcctgcagcgaggccctcctggagcgcttcatcatcttcagccagagacgcggggcaaagacggtgcgctatgccctgtgctccctctcccagggcaccctacagtggatagaagacactctgtatgccaacgtggacttcttcaagctcttccgtgtgcttcccacactcctagacagccgttctcaaggtatcaatctgagatcttggggaggaatattatctgatatgtcaccaagaattcaagagtttatccatcggccgagtatgcaggacttgctgtgggtgaccaggcccctcatgcagaatggtggtccagagacctttacaaagctgatgggcatcctgtctgacctcctgtgtggctaccccgagggaggtggctctcgggtgctctccttcaactggtatgaagacaataactataaggcctttctggggattgactccacaaggaaggatcctatctattcttatgacagaagaacaacatccttttgtaatgcattgatccagagcctggagtcaaatcctttaaccaaaatcgcttggagggcggcaaagcctttgctgatgggaaaaatcctgtacactcctgattcacctgcagcacgaaggatactgaagaatgccaactcaacttttgaagaactggaacacgttaggaagttggtcaaagcctgggaagaagtagggccccagatctggtacttctttgacaacagcacacagatgaacatgatcagagataccctggggaacccaacagtaaaagactttttgaataggcagcttggtgaagaaggtattactgctgaagccatcctaaacttcctctacaagggccctcgggaaagccaggctgacgacatggccaacttcgactggagggacatatttaacatcactgatcgcaccctccgcctggtcaatcaatacctggagtgcttggtcctggataagtttgaaagctacaatgatgaaactcagctcacccaacgtgccctctctctactggaggaaaacatgttctgggccggagtggtattccctgacatgtatccctggaccagctctctaccaccccacgtgaagtataagatccgaatggacatagacgtggtggagaaaaccaataagattaaagacaggtattgggattctggtcccagagctgatcccgtggaagatttccggtacatctggggcgggtttgcctatctgcaggacatggttgaacaggggatcacaaggagccaggtgcaggcggaggctccagttggaatctacctccagcagatgccctacccctgcttcgtggacgattctttcatgatcatcctgaaccgctgtttccctatcttcatggtgctggcatggatctactctgtctccatgactgtgaagagcatcgtcttggagaaggagttgcgactgaaggagaccttgaaaaatcagggtgtctccaatgcagtgatttggtgtacctggttcctggacagcttctccatcatgtcgatgagcatcttcctcctgacgatattcatcatgcatggaagaatcctacattacagcgacccattcatcctcttcctgttcttgttggctttctccactgccaccatcatgctgtgctttctgctcagcaccttcttctccaaggccagtctggcagcagcctgtagtggtgtcatctatttcaccctctacctgccacacatcctgtgcttcgcctggcaggaccgcatgaccgctgagctgaagaaggctgtgagcttactgtctccggtggcatttggatttggcactgagtacctggttcgctttgaagagcaaggcctggggctgcagtggagcaacatcgggaacagtcccacggaaggggacgaattcagcttcctgctgtccatgcagatgatgctccttgatgctgctgtctatggcttactcgcttggtaccttgatcaggtgtttccaggagactatggaaccccacttccttggtactttcttctacaagagtcgtattggcttggcggtgaagggtgttcaaccagagaagaaagagccctggaaaagaccgagcccctaacagaggaaacggaggatccagagcacccagaaggaatacacgactccttctttgaacgtgagcatccagggtgggttcctggggtatgcgtgaagaatctggtaaagatttttgagccctgtggccggccagctgtggaccgtctgaacatcaccttctacgagaaccagatcaccgcattcctgggccacaatggagctgggaaaaccaccaccttgtccatcctgacgggtctgttgccaccaacctctgggactgtgctcgttgggggaagggacattgaaaccagcctggatgcagtccggcagagccttggcatgtgtccacagcacaacatcctgttccaccacctcacggtggctgagcacatgctgttctatgcccagctgaaaggaaagtcccaggaggaggcccagctggagatggaagccatgttggaggacacaggcctccaccacaagcggaatgaagaggctcaggacctatcaggtggcatgcagagaaagctgtcggttgccattgcctttgtgggagatgccaaggtggtgattctggacgaacccacctctggggtggacccttactcgagacgctcaatctgggatctgctcctgaagtatcgctcaggcagaaccatcatcatgtccactcaccacatggacgaggccgacctccttggggaccgcattgccatcattgcccagggaaggctctactgctcaggcaccccactcttcctgaagaactgctttggc

SEQ ID NO: 28 - DNA, 2448 bp, synthetic construct
  source 1..2448: mol_type = other DNA
acacagctggtcctccagcatgtgcaggcgctgctggtcaagagattccaacacaccatccgcagccacaaggacttcctggcgcagatcgtgctcccggctacctttgtgtttttggctctgatgctttctattgttatccctccttttggcgaataccccgctttgacccttcacccctggatatatgggcagcagtacaccttcttcagcatggatgaaccaggcagtgagcagttcacggtacttgcagacgtcctcctgaataagccaggctttggcaaccgctgcctgaaggaagggtggcttccggagtacccctgtggcaactcaacaccctggaagactccttctgtgtccccaaacatcacccagctgttccagaagcagaaatggacacaggtcaacccttcaccatcctgcaggtgcagcaccagggagaagctcaccatgctgccagagtgccccgagggtgccgggggcctcccgcccccccagagaacacagcgcagcacggaaattctacaagacctgacggacaggaacatctccgacttcttggtaaaaacgtatcctgctcttataagaagcagcttaaagagcaaattctgggtcaatgaacagaggtatggaggaatttccattggaggaaagctcccagtcgtccccatcacgggggaagcacttgttgggtttttaagcgaccttggccggatcatgaatgtgagcgggggccctatcactagagaggcctctaaagaaatacctgatttccttaaacatctagaaactgaagacaacattaaggtgtggtttaataacaaaggctggcatgccctggtcagctttctcaatgtggcccacaacgccatcttacgggccagcctgcctaaggacaggagccccgaggagtatggaatcaccgtcattagccaacccctgaacctgaccaaggagcagctctcagagattacagtgctgaccacttcagtggatgctgtggttgccatctgcgtgattttctccatgtccttcgtcccagccagctttgtcctttatttgatccaggagcgggtgaacaaatccaagcacctccagtttatcagtggagtgagccccaccacctactgggtgaccaacttcctctgggacatcatgaattattccgtgagtgctgggctggtggtgggcatcttcatcgggtttcagaagaaagcctacacttctccagaaaaccttcctgcccttgtggcactgctcctgctgtatggatgggcggtcattcccatgatgtacccagcatccttcctgtttgatgtccccagcacagcctatgtggctttatcttgtgctaatctgttcatcggcatcaacagcagtgctattaccttcatcttggaattatttgagaataaccggacgctgctcaggttcaacgccgtgctgaggaagctgctcattgtcttcccccacttctgcctgggccggggcctcattgaccttgcactgagccaggctgtgacagatgtctatgcccggtttggtgaggagcactctgcaaatccgttccactgggacctgattgggaagaacctgtttgccatggtggtggaaggggtggtgtacttcctcctgaccctgctggtccagcgccacttcttcctctcccaatggattgccgagcccactaaggagcccattgttgatgaagatgatgatgtggctgaagaaagacaaagaattattactggtggaaataaaactgacatcttaaggctacatgaactaaccaagatttatccaggcacctccagcccagcagtggacaggctgtgtgtcggagttcgccctggagagtgctttggcctcctgggagtgaatggtgccggcaaaacaaccacattcaagatgctcactggggacaccacagtgacctcaggggatgccaccgtagcaggcaagagtattttaaccaatatttctgaagtccatcaaaatatgggctactgtcctcagtttgatgcaattgatgagctgctcacaggacgagaacatctttacctttatgcccggcttcgaggtgtaccagcagaagaaatcgaaaaggttgcaaactggagtattaagagcctgggcctgactgtctacgccgactgcctggctggcacgtacagtgggggcaacaagcggaaactctccacagccatcgcactcattggctgcccaccgctggtgctgctggatgagcccaccacagggatggacccccaggcacgccgcatgctgtggaacgtcatcgtgagcatcatcagagaagggagggctgtggtcctcacatcccacagcatggaagaatgtgaggcactgtgtacccggctggccatcatggtaaagggcgcctttcgatgtatgggcaccattcagcatctcaagtccaaatttggagat

SEQ ID NO: 29 - DNA, 681 bp, synthetic construct
  source 1..681: mol_type = other DNA
gataagacccacacctgccccccatgtcctgctcctgagctgctgggcggacctagcgttttcctgtttccccccaaaccaaaggacaccctgatgatcagccggacccctgaggtgacatgcgtggtggtggacgtgtcccacgaggaccctgaggtgaagttcaactggtatgtggacggcgtggaagtgcacaatgccaagaccaagcccagagaggagcagtacaacagcacctacagagtggtcagcgtgcttacagtcctccatcaggattggctgaatggcaaggaatacaagtgcaaggtgtctaacaaggccctgcccgcccctatcgagaagaccatcagcaaggctaagggccaacctcgggaacctcaggtctacaccctgcctccaagcagagaggaaatgaccaaaaaccaggtgtccctgtggtgcctggtgaagggattttaccccagcgacatcgccgtggaatgggagagcaacggccagcctgaaaacaactacaagacaacacctcctgtgctggacagcgacggcagcttcttcctgtactctaaactgacagtggataagtccagatggcagcagggcaacgtgttcagctgtagcgtgatgcacgaggccctgcacaaccactacacccagaagagcctgtctctgagccctggcaaa

SEQ ID NO: 30 - DNA, 681 bp, synthetic construct
  source 1..681: mol_type = other DNA
gataagacacacacctgtcctccatgtcctgcccctgagctgctgggcggaccttctgtctttctgttcccccccaagcctaaggacaccctggaagccagccggacccctgaggtgacctgcgtggtcgtcgacgtgtcccacgaggaccccgaggtgaagttcaactggtacgtggatggcgttgaggtgcacaacgccaaaaccaagcccagagaggaacagtacaacagcacctaccgggtggtgtccgtgctgaccgtgctccaccaggactggctgaacggcaaggaatacaagtgcaaggtgtccaacaaggccctgcccgctcctatcgagaagaccatcagcaaggccaagggccagcctagagaacctcaggtgtacaccctgcctccaagcagagaggaaatgacaaagaaccaggtgtctctgagctgcgccgtgaaaggcttctaccccagcgatatcgccgtggaatgggagagcaatggccaacctgaaaacaactacaagaccacaccacctgtgctggacagcgacggaagctttttcctggtgtccaagctgacagtggacaagagcagatggcagcagggcaacgtgttcagctgcagcgtgatgcacgaggccctgcataatgcttatacacagaaaagcctgagcctgtctcctggaaaa

SEQ ID NO: 31 - DNA, 4737 bp, synthetic construct
  source 1..4737: mol_type = other DNA
atgggattcgtgcggcagatccagcttctgctctggaagaattggaccctgcgtaaacggcagaagattagatttgtggtggagctggtgtggcctctgagcctgttcttggtgctgatctggctgcgaaacgccaaccctctgtactcccaccatgagtgtcacttccctaacaaggccatgccttctgctggcatgctgccttggctgcagggcatcttctgcaacgtgaacaacccctgcttccagagccccacccctggagagtctcccggcatcgtcagtaactacaacaactccatcctcgccagagtgtacagagatttccaggagctgctgatgaacgcccctgagtctcaacacctggggagaatctggaccgagctccatatactgtcacagttcatggataccctacggacccaccccgaacggatcgccggcagaggcattagaatccgggatatccttaaggacgaagagacactgactctttttctgattaagaatatcggattgtctgattcggtggtgtacctgctgatcaacagccaggtgagacctgagcagttcgcccacggcgtgcctgacttagcgctgaaggacattgcctgctctgaggccttgctggaaagattcatcatcttctctcagcggcggggggccaagacagttcggtacgccctgtgcagcctgagccagggcaccttgcagtggatcgaagacaccctgtatgctaacgtggacttctttaaactgtttagagtgttgccaaccttactggacagccggagccagggcatcaacctgagatcctggggtggaatcctgagcgatatgagccccagaatccaggagttcatccaccggcctagcatgcaggacttgctgtgggtgactcgtcccctgatgcaaaacggaggaccagaaacatttacaaagcttatgggcatcctgagcgacctcttgtgcggctaccctgagggcggcggcagccgggtgttaagctttaactggtacgaggacaacaactacaaggccttccttggtatcgatagcacacgaaaggacccaatctacagctacgaccgtagaacaaccagtttctgcaacgccctgatccagtcccttgaatctaatcctttgacaaagatcgcttggcgggccgccaagcctctgctgatgggcaagatcctgtacacccctgacagccctgccgccagaagaatcctaaagaatgccaacagcactttcgaggaactcgaacacgtgcggaagctggtcaaagcctgggaggaggtgggccctcaaatctggtacttcttcgataactccacccagatgaacatgatcagagacaccttgggaaatccgaccgtgaaggacttcctgaatagacagctaggtgaggagggaatcaccgccgaggccatcctgaactttctgtacaaaggccctcgggagtcccaggctgatgacatggccaattttgactggagagacatattcaacatcacagaccgtacccttagactggtgaaccagtacctggaatgcttagtcctggataagttcgaaagctacaacgacgagacccagctgacccaacgggcactgtctctactggaggagaatatgttctgggccggtgtggtgttccctgacatgtacccctggacaagcagcctgccacctcacgtgaaatacaagatccggatggacattgacgtggtggaaaagacaaacaagatcaaggacagatactgggacagcggacctagggccgatcctgtggaggatttccggtacatctggggtggcttcgcttacctgcaggacatggtggaacagggcatcacgagaagccaggtgcaggctgaggcccctgtgggaatctacctccaacagatgccctacccctgcttcgtggacgacagcttcatgatcatcctgaatagatgtttcccaatcttcatggtgctggcctggatctacagcgtgtccatgactgtgaagtccatcgtgctggagaaggagctgcggctaaaagagactctgaagaatcagggcgtgagcaacgccgtaatctggtgcacctggttcctggactccttctccatcatgagcatgagcatcttcctactgacaatctttatcatgcacggcagaattctgcactacagcgaccctttcatcctgtttctttttttgctggctttcagcaccgccaccatcatgctgtgcttcctgttaagcaccttcttctcaaaggccagcctagctgcagcatgctccggcgtcatctactttactttatacctgccccacatcctgtgtttcgcctggcaggacagaatgacagccgagctgaaaaaggccgtatccctgttgagccccgtggccttcgggtttggaaccgagtacctggtacggttcgaggaacaaggcctgggcctgcagtggtccaacatcggcaactcgccgaccgagggcgacgaattcagcttcctgctgtccatgcagatgatgctgctggatgccgcagtgtatggcctcctggcttggtacttggaccaggtgttccccggcgactacgggactccactgccatggtactttctgctgcaggagagctactggctgggcggcgagggctgcagcaccagagaggaaagagccctggagaagacagagcctctgactgaagaaaccgaagaccctgagcaccctgaggggatacacgactcttttttcgagagggaacatcctggatgggtccctggcgtttgcgtgaagaacctggtgaagatcttcgagccttgtggcaggccagccgtggatagactgaatatcaccttctacgagaaccagatcaccgccttcctgggccacaacggcgcgggaaagaccacaactctgagcatcctgaccggactgctgcctccaacttccggcaccgtgctcgtcggcggcagggacatcgagaccagtctggacgccgtgagacagagcctcggcatgtgccctcagcacaatatcctgtttcaccacttaaccgttgcagaacacatgctgttctacgcccagttaaaaggcaagtcgcaggaggaggcccagctggagatggaagcaatgctcgaagatacaggcctgcaccataagagaaacgaagaggcccaggatctctccggcggcatgcagagaaaactgagcgtagccatcgccttcgtgggagatgcaaaggtggtaatcctagatgagcctacatctggggtggacccgtacagccggcgcagtatttgggatttactgctgaagtacagaagcggtagaaccatcatcatgtctacccaccacatggacgaggctgatctgctgggagatcggatcgccataatcgcccagggaagactgtattgcagcggcacaccactgttcctcaaaaactgctttgggacgggactgtacctgacgctggtccggaaaatgaagaacatccagtcccagagaaagggctctgaagggacctgttcttgcagctctaagggcttcagtaccacctgccctgcccacgtggacgacctgactcccgaacaggtgctggacggcgatgtgaacgagctgatggacgtggtgctgcatcacgtacccgaagccaagctggttgaatgcatcggccaggagctcattttccttcttcctaacaagaacttcaagcacagagcttatgcctctctgttcagggaactggaggaaaccctagccgacctgggtctgtctagcttcggcatctctgacacacctctggaggagatctttctgaaagtgactgaggattctgatagcggaccactgttcgccggaggcgctcagcagaagagagaaaacgtcaatcctagacacccttgtctgggaccgagagagaaggccggccagacccctcaagattccaatgtgtgtagccctggcgcccccgctgctcacccagagggccagcctcctcctgaacctgaatgccccggcccccagctgaacaccggctctggcagcggcagcgataagacccacacctgccccccatgtcctgctcctgagctgctgggcggacctagcgttttcctgtttccccccaaaccaaaggacaccctgatgatcagccggacccctgaggtgacatgcgtggtggtggacgtgtcccacgaggaccctgaggtgaagttcaactggtatgtggacggcgtggaagtgcacaatgccaagaccaagcccagagaggagcagtacaacagcacctacagagtggtcagcgtgcttacagtcctccatcaggattggctgaatggcaaggaatacaagtgcaaggtgtctaacaaggccctgcccgcccctatcgagaagaccatcagcaaggctaagggccaacctcgggaacctcaggtctacaccctgcctccaagcagagaggaaatgaccaaaaaccaggtgtccctgtggtgcctggtgaagggattttaccccagcgacatcgccgtggaatgggagagcaacggccagcctgaaaacaactacaagacaacacctcctgtgctggacagcgacggcagcttcttcctgtactctaaactgacagtggataagtccagatggcagcagggcaacgtgttcagctgtagcgtgatgcacgaggccctgcacaaccactacacccagaagagcctgtctctgagccctggcaaa

SEQ ID NO: 32 - DNA, 3480 bp, synthetic construct
  source 1..3480: mol_type = other DNA
atgactcagctggtcctgcagcacgtgcaggccctgctggtgaagcgcttccagcacacaatccgcagtcataaagacttcctcgctcagatcgtgctcccggctacattcgtgtttctggccctcatgctgtctatcgtgatcccacctttcggcgaataccctgcgctgaccctgcacccctggatatacggtcagcaatacacctttttcagcatggacgagcccggaagcgagcagttcaccgtgctggccgatgtgctgctgaacaagcctggcttcggcaaccggtgcctgaaagaaggatggctgccagagtacccctgcggcaatagcacaccttggaagacccctagcgtgtcccctaacatcacccagctgtttcaaaaacagaaatggacccaagtgaatccttcaccttcatgcagatgttctacacgtgaaaagctgaccatgttacccgagtgtcctgaaggagctggcggccttcctcctccccagaggacccagagaagcaccgaaatcctgcaggacctgacagaccggaacatctccgactttcttgtcaagacctaccctgccctgattaggagtagcctgaaatctaagttttgggttaatgaacagcggtacggcggcatcagcatcggcggtaagctgcccgtggtgcctattacaggcgaggccctggtgggcttcctcagtgatttgggacggataatgaacgtgagtggcggcccaatcacacgggaagccagcaaagagatccctgatttcctgaagcacctggaaacagaggataatataaaggtgtggttcaacaacaaaggctggcacgccctggtgagtttcctcaacgtagcccacaacgctatcctgagagcctctctacctaaggacagaagccccgaagagtacggcattaccgtgatcagccagcccctaaacctgacaaaggaacagctgagcgagattaccgtcctgacaacctccgttgacgcggtggtggcgatctgcgtgatcttttctatgagcttcgtgcctgccagcttcgtgctgtacctgatccaggagagagtgaacaagagcaagcacctgcaatttatttctggcgtgagcccaaccacctactgggtgaccaacttcctgtgggacatcatgaactacagcgtgtctgccggcctggtggtaggcatcttcatcggcttccagaagaaggcctacacctctcctgagaatctgcctgctctcgtggccctgctgctgctgtacggctgggccgtgatccccatgatgtaccccgctagcttcttatttgacgtgccctcaacagcatacgtggccttatcctgcgccaacctgtttataggaatcaattctagcgccatcacgttcatcctagaactgttcgagaacaaccggacactgctgcgattcaacgccgtcctgcggaagctcctgattgtgttccctcatttctgtctgggcagagggctgatcgacctggccctgagccaagccgtgaccgatgtgtacgcgagattcggcgaggagcactccgccaaccctttccactgggacctgatcggcaagaatctgttcgccatggttgtggagggtgtggtgtacttcctgcttacactgctggtgcagagacacttcttcctgtcccagtggattgccgaacccaccaaggaacccatcgtcgacgaggatgacgacgtggccgaggagagacagagaatcatcaccggcgggaacaaaaccgacatcctgagactccacgagctgacaaagatctatcctggcacaagcagccccgccgtggatcggctgtgtgtgggcgtcagacctggcgagtgcttcggcctgctgggcgtgaacggcgccggcaagaccacaaccttcaagatgctgaccggcgacaccacggtgacctccggcgacgccacagtggccggcaaaagcatcctcacaaacatctccgaagtgcaccagaacatgggctactgcccccagtttgatgctatagacgagctgttgaccggtagagaacacctgtacctgtacgccagactgagaggcgtgcctgctgaagagatcgaaaaggtggcaaactggagcatcaagtcactgggcctgacagtctacgccgactgcctggccggcacgtactctggcggcaataagcggaaactgagcaccgccattgccttgattggatgtccgcctctggtgctgctggacgagccgacaacaggcatggacccccaagcccggagaatgctgtggaacgtgatcgtgagcataatcagagagggcagagccgtggttttgacttctcacagcatggaagaatgtgaagcgctctgcacccggcttgccatcatggtcaaaggcgccttccggtgcatgggcaccattcagcacctgaagtccaagttcggcgacggctacatcgtgacaatgaagatcaaatctcccaaggacgacctgcttccagatctgaaccctgtggaacagttcttccagggaaatttccctggaagcgtgcagagagagagacactacaatatgctgcagtttcaggtaagcagcagcagccttgctcggatctttcagctgctgcttagccacaaggactctctgctgatcgaagagtacagcgtgacccagacaacgcttgatcaggtgttcgtgaacttcgccaagcagcaaaccgagagccatgatctgcctcttcacccacgagctgccggcgccagcagacaggcccaggactctggcagcggcagcgataagacacacacctgtcctccatgtcctgcccctgagctgctgggcggaccttctgtctttctgttcccccccaagcctaaggacaccctggaagccagccggacccctgaggtgacctgcgtggtcgtcgacgtgtcccacgaggaccccgaggtgaagttcaactggtacgtggatggcgttgaggtgcacaacgccaaaaccaagcccagagaggaacagtacaacagcacctaccgggtggtgtccgtgctgaccgtgctccaccaggactggctgaacggcaaggaatacaagtgcaaggtgtccaacaaggccctgcccgctcctatcgagaagaccatcagcaaggccaagggccagcctagagaacctcaggtgtacaccctgcctccaagcagagaggaaatgacaaagaaccaggtgtctctgagctgcgccgtgaaaggcttctaccccagcgatatcgccgtggaatgggagagcaatggccaacctgaaaacaactacaagaccacaccacctgtgctggacagcgacggaagctttttcctggtgtccaagctgacagtggacaagagcagatggcagcagggcaacgtgttcagctgcagcgtgatgcacgaggccctgcataatgcttatacacagaaaagcctgagcctgtctcctggaaaatga

SEQ ID NO: 33 - DNA, 3480 bp, synthetic construct
  source 1..3480: mol_type = other DNA
atggataagacacacacctgtcctccatgtcctgcccctgagctgctgggcggaccttctgtctttctgttcccccccaagcctaaggacaccctggaagccagccggacccctgaggtgacctgcgtggtcgtcgacgtgtcccacgaggaccccgaggtgaagttcaactggtacgtggatggcgttgaggtgcacaacgccaaaaccaagcccagagaggaacagtacaacagcacctaccgggtggtgtccgtgctgaccgtgctccaccaggactggctgaacggcaaggaatacaagtgcaaggtgtccaacaaggccctgcccgctcctatcgagaagaccatcagcaaggccaagggccagcctagagaacctcaggtgtacaccctgcctccaagcagagaggaaatgacaaagaaccaggtgtctctgagctgcgccgtgaaaggcttctaccccagcgatatcgccgtggaatgggagagcaatggccaacctgaaaacaactacaagaccacaccacctgtgctggacagcgacggaagctttttcctggtgtccaagctgacagtggacaagagcagatggcagcagggcaacgtgttcagctgcagcgtgatgcacgaggccctgcataatgcttatacacagaaaagcctgagcctgtctcctggaaaatctggcagcggcagcactcagctggtcctgcagcacgtgcaggccctgctggtgaagcgcttccagcacacaatccgcagtcataaagacttcctcgctcagatcgtgctcccggctacattcgtgtttctggccctcatgctgtctatcgtgatcccacctttcggcgaataccctgcgctgaccctgcacccctggatatacggtcagcaatacacctttttcagcatggacgagcccggaagcgagcagttcaccgtgctggccgatgtgctgctgaacaagcctggcttcggcaaccggtgcctgaaagaaggatggctgccagagtacccctgcggcaatagcacaccttggaagacccctagcgtgtcccctaacatcacccagctgtttcaaaaacagaaatggacccaagtgaatccttcaccttcatgcagatgttctacacgtgaaaagctgaccatgttacccgagtgtcctgaaggagctggcggccttcctcctccccagaggacccagagaagcaccgaaatcctgcaggacctgacagaccggaacatctccgactttcttgtcaagacctaccctgccctgattaggagtagcctgaaatctaagttttgggttaatgaacagcggtacggcggcatcagcatcggcggtaagctgcccgtggtgcctattacaggcgaggccctggtgggcttcctcagtgatttgggacggataatgaacgtgagtggcggcccaatcacacgggaagccagcaaagagatccctgatttcctgaagcacctggaaacagaggataatataaaggtgtggttcaacaacaaaggctggcacgccctggtgagtttcctcaacgtagcccacaacgctatcctgagagcctctctacctaaggacagaagccccgaagagtacggcattaccgtgatcagccagcccctaaacctgacaaaggaacagctgagcgagattaccgtcctgacaacctccgttgacgcggtggtggcgatctgcgtgatcttttctatgagcttcgtgcctgccagcttcgtgctgtacctgatccaggagagagtgaacaagagcaagcacctgcaatttatttctggcgtgagcccaaccacctactgggtgaccaacttcctgtgggacatcatgaactacagcgtgtctgccggcctggtggtaggcatcttcatcggcttccagaagaaggcctacacctctcctgagaatctgcctgctctcgtggccctgctgctgctgtacggctgggccgtgatccccatgatgtaccccgctagcttcttatttgacgtgccctcaacagcatacgtggccttatcctgcgccaacctgtttataggaatcaattctagcgccatcacgttcatcctagaactgttcgagaacaaccggacactgctgcgattcaacgccgtcctgcggaagctcctgattgtgttccctcatttctgtctgggcagagggctgatcgacctggccctgagccaagccgtgaccgatgtgtacgcgagattcggcgaggagcactccgccaaccctttccactgggacctgatcggcaagaatctgttcgccatggttgtggagggtgtggtgtacttcctgcttacactgctggtgcagagacacttcttcctgtcccagtggattgccgaacccaccaaggaacccatcgtcgacgaggatgacgacgtggccgaggagagacagagaatcatcaccggcgggaacaaaaccgacatcctgagactccacgagctgacaaagatctatcctggcacaagcagccccgccgtggatcggctgtgtgtgggcgtcagacctggcgagtgcttcggcctgctgggcgtgaacggcgccggcaagaccacaaccttcaagatgctgaccggcgacaccacggtgacctccggcgacgccacagtggccggcaaaagcatcctcacaaacatctccgaagtgcaccagaacatgggctactgcccccagtttgatgctatagacgagctgttgaccggtagagaacacctgtacctgtacgccagactgagaggcgtgcctgctgaagagatcgaaaaggtggcaaactggagcatcaagtcactgggcctgacagtctacgccgactgcctggccggcacgtactctggcggcaataagcggaaactgagcaccgccattgccttgattggatgtccgcctctggtgctgctggacgagccgacaacaggcatggacccccaagcccggagaatgctgtggaacgtgatcgtgagcataatcagagagggcagagccgtggttttgacttctcacagcatggaagaatgtgaagcgctctgcacccggcttgccatcatggtcaaaggcgccttccggtgcatgggcaccattcagcacctgaagtccaagttcggcgacggctacatcgtgacaatgaagatcaaatctcccaaggacgacctgcttccagatctgaaccctgtggaacagttcttccagggaaatttccctggaagcgtgcagagagagagacactacaatatgctgcagtttcaggtaagcagcagcagccttgctcggatctttcagctgctgcttagccacaaggactctctgctgatcgaagagtacagcgtgacccagacaacgcttgatcaggtgttcgtgaacttcgccaagcagcaaaccgagagccatgatctgcctcttcacccacgagctgccggcgccagcagacaggcccaggactga

SEQ ID NO: 34 - protein, 1579 aa, synthetic construct
MGFVRQIQLLLWKNWTLRKRQKIRFVVELVWPLSLFLVLIWLRNANPLYSHHECHFPNKAMPSAGMLPWLQGIFCNVNNPCFQSPTPGESPGIVSNYNNSILARVYRDFQELLMNAPESQHLGRIWTELHILSQFMDTLRTHPERIAGRGIRIRDILKDEETLTLFLIKNIGLSDSVVYLLINSQVRPEQFAHGVPDLALKDIACSEALLERFIIFSQRRGAKTVRYALCSLSQGTLQWIEDTLYANVDFFKLFRVLPTLLDSRSQGINLRSWGGILSDMSPRIQEFIHRPSMQDLLWVTRPLMQNGGPETFTKLMGILSDLLCGYPEGGGSRVLSFNWYEDNNYKAFLGIDSTRKDPIYSYDRRTTSFCNALIQSLESNPLTKIAWRAAKPLLMGKILYTPDSPAARRILKNANSTFEELEHVRKLVKAWEEVGPQIWYFFDNSTQMNMIRDTLGNPTVKDFLNRQLGEEGITAEAILNFLYKGPRESQADDMANFDWRDIFNITDRTLRLVNQYLECLVLDKFESYNDETQLTQRALSLLEENMFWAGVVFPDMYPWTSSLPPHVKYKIRMDIDVVEKTNKIKDRYWDSGPRADPVEDFRYIWGGFAYLQDMVEQGITRSQVQAEAPVGIYLQQMPYPCFVDDSFMIILNRCFPIFMVLAWIYSVSMTVKSIVLEKELRLKETLKNQGVSNAVIWCTWFLDSFSIMSMSIFLLTIFIMHGRILHYSDPFILFLFLLAFSTATIMLCFLLSTFFSKASLAAACSGVIYFTLYLPHILCFAWQDRMTAELKKAVSLLSPVAFGFGTEYLVRFEEQGLGLQWSNIGNSPTEGDEFSFLLSMQMMLLDAAVYGLLAWYLDQVFPGDYGTPLPWYFLLQESYWLGGEGCSTREERALEKTEPLTEETEDPEHPEGIHDSFFEREHPGWVPGVCVKNLVKIFEPCGRPAVDRLNITFYENQITAFLGHNGAGKTTTLSILTGLLPPTSGTVLVGGRDIETSLDAVRQSLGMCPQHNILFHHLTVAEHMLFYAQLKGKSQEEAQLEMEAMLEDTGLHHKRNEEAQDLSGGMQRKLSVAIAFVGDAKVVILDEPTSGVDPYSRRSIWDLLLKYRSGRTIIMSTHHMDEADLLGDRIAIIAQGRLYCSGTPLFLKNCFGTGLYLTLVRKMKNIQSQRKGSEGTCSCSSKGFSTTCPAHVDDLTPEQVLDGDVNELMDVVLHHVPEAKLVECIGQELIFLLPNKNFKHRAYASLFRELEETLADLGLSSFGISDTPLEEIFLKVTEDSDSGPLFAGGAQQKRENVNPRHPCLGPREKAGQTPQDSNVCSPGAPAAHPEGQPPPEPECPGPQLNTGSGSGSDKTHTCPPCPAPELLGGPSVFLFPPKPKDTLEASRTPEVTCVVVDVSHEDPEVKFNWYVDGVEVHNAKTKPREEQYNSTYRVVSVLTVLHQDWLNGKEYKCKVSNKALPAPIEKTISKAKGQPREPQVYTLPPSREEMTKNQVSLSCAVKGFYPSDIAVEWESNGQPENNYKTTPPVLDSDGSFFLVSKLTVDKSRWQQGNVFSCSVMHEALHNAYTQKSLSLSPGK

SEQ ID NO: 35 - protein, 1160 aa, synthetic construct
MGFVRQIQLLLWKNWTLRKRQKIRFVVELVWPLSLFLVLIWLRNANPLYSHHECHFPNKAMPSAGMLPWLQGIFCNVNNPCFQSPTPGESPGIVSNYNNSILARVYRDFQELLMNAPESQHLGRIWTELHILSQFMDTLRTHPERIAGRGIRIRDILKDEETLTLFLIKNIGLSDSVVYLLINSQVRPEQFAHGVPDLALKDIACSEALLERFIIFSQRRGAKTVRYALCSLSQGTLQWIEDTLYANVDFFKLFRVLPTLLDSRSQGINLRSWGGILSDMSPRIQEFIHRPSMQDLLWVTRPLMQNGGPETFTKLMGILSDLLCGYPEGGGSRVLSFNWYEDNNYKAFLGIDSTRKDPIYSYDRRTTSFCNALIQSLESNPLTKIAWRAAKPLLMGKILYTPDSPAARRILKNANSTFEELEHVRKLVKAWEEVGPQIWYFFDNSTQMNMIRDTLGNPTVKDFLNRQLGEEGITAEAILNFLYKGPRESQADDMANFDWRDIFNITDRTLRLVNQYLECLVLDKFESYNDETQLTQRALSLLEENMFWAGVVFPDMYPWTSSLPPHVKYKIRMDIDVVEKTNKIKDRYWDSGPRADPVEDFRYIWGGFAYLQDMVEQGITRSQVQAEAPVGIYLQQMPYPCFVDDSFMIILNRCFPIFMVLAWIYSVSMTVKSIVLEKELRLKETLKNQGVSNAVIWCTWFLDSFSIMSMSIFLLTIFIMHGRILHYSDPFILFLFLLAFSTATIMLCFLLSTFFSKASLAAACSGVIYFTLYLPHILCFAWQDRMTAELKKAVSLLSPVAFGFGTEYLVRFEEQGLGLQWSNIGNSPTEGDEFSFLLSMQMMLLDAAVYGLLAWYLDQVFPGDYGTPLPWYFLLQESYWLGGEGCSTREERALEKTEPLTEETEDPEHPEGIHDSFFEREHPGWVPGVCVKNLVKIFEPCGRPAVDRLNITFYENQITAFLGHNGAGKTTTLSILTGLLPPTSGTVLVGGRDIETSLDAVRQSLGMCPQHNILFHHLTVAEHMLFYAQLKGKSQEEAQLEMEAMLEDTGLHHKRNEEAQDLSGGMQRKLSVAIAFVGDAKVVILDEPTSGVDPYSRRSIWDLLLKYRSGRTIIMSTHHMDEADLLGDRIAIIAQGRLYCSGTPLFLKNCFGTGLYLTLV

SEQ ID NO: 36 - protein, 1220 aa, synthetic construct
MGFVRQIQLLLWKNWTLRKRQKIRFVVELVWPLSLFLVLIWLRNANPLYSHHECHFPNKAMPSAGMLPWLQGIFCNVNNPCFQSPTPGESPGIVSNYNNSILARVYRDFQELLMNAPESQHLGRIWTELHILSQFMDTLRTHPERIAGRGIRIRDILKDEETLTLFLIKNIGLSDSVVYLLINSQVRPEQFAHGVPDLALKDIACSEALLERFIIFSQRRGAKTVRYALCSLSQGTLQWIEDTLYANVDFFKLFRVLPTLLDSRSQGINLRSWGGILSDMSPRIQEFIHRPSMQDLLWVTRPLMQNGGPETFTKLMGILSDLLCGYPEGGGSRVLSFNWYEDNNYKAFLGIDSTRKDPIYSYDRRTTSFCNALIQSLESNPLTKIAWRAAKPLLMGKILYTPDSPAARRILKNANSTFEELEHVRKLVKAWEEVGPQIWYFFDNSTQMNMIRDTLGNPTVKDFLNRQLGEEGITAEAILNFLYKGPRESQADDMANFDWRDIFNITDRTLRLVNQYLECLVLDKFESYNDETQLTQRALSLLEENMFWAGVVFPDMYPWTSSLPPHVKYKIRMDIDVVEKTNKIKDRYWDSGPRADPVEDFRYIWGGFAYLQDMVEQGITRSQVQAEAPVGIYLQQMPYPCFVDDSFMIILNRCFPIFMVLAWIYSVSMTVKSIVLEKELRLKETLKNQGVSNAVIWCTWFLDSFSIMSMSIFLLTIFIMHGRILHYSDPFILFLFLLAFSTATIMLCFLLSTFFSKASLAAACSGVIYFTLYLPHILCFAWQDRMTAELKKAVSLLSPVAFGFGTEYLVRFEEQGLGLQWSNIGNSPTEGDEFSFLLSMQMMLLDAAVYGLLAWYLDQVFPGDYGTPLPWYFLLQESYWLGGEGCSTREERALEKTEPLTEETEDPEHPEGIHDSFFEREHPGWVPGVCVKNLVKIFEPCGRPAVDRLNITFYENQITAFLGHNGAGKTTTLSILTGLLPPTSGTVLVGGRDIETSLDAVRQSLGMCPQHNILFHHLTVAEHMLFYAQLKGKSQEEAQLEMEAMLEDTGLHHKRNEEAQDLSGGMQRKLSVAIAFVGDAKVVILDEPTSGVDPYSRRSIWDLLLKYRSGRTIIMSTHHMDEADLLGDRIAIIAQGRLYCSGTPLFLKNCFGTGLYLTLVRKMKNIQSQRKGSEGTCSCSSKGFSTTCPAHVDDLTPEQVLDGDVNELMDVVLHHVPEAK

SEQ ID NO: 37 - protein, 1280 aa, synthetic construct
MGFVRQIQLLLWKNWTLRKRQKIRFVVELVWPLSLFLVLIWLRNANPLYSHHECHFPNKAMPSAGMLPWLQGIFCNVNNPCFQSPTPGESPGIVSNYNNSILARVYRDFQELLMNAPESQHLGRIWTELHILSQFMDTLRTHPERIAGRGIRIRDILKDEETLTLFLIKNIGLSDSVVYLLINSQVRPEQFAHGVPDLALKDIACSEALLERFIIFSQRRGAKTVRYALCSLSQGTLQWIEDTLYANVDFFKLFRVLPTLLDSRSQGINLRSWGGILSDMSPRIQEFIHRPSMQDLLWVTRPLMQNGGPETFTKLMGILSDLLCGYPEGGGSRVLSFNWYEDNNYKAFLGIDSTRKDPIYSYDRRTTSFCNALIQSLESNPLTKIAWRAAKPLLMGKILYTPDSPAARRILKNANSTFEELEHVRKLVKAWEEVGPQIWYFFDNSTQMNMIRDTLGNPTVKDFLNRQLGEEGITAEAILNFLYKGPRESQADDMANFDWRDIFNITDRTLRLVNQYLECLVLDKFESYNDETQLTQRALSLLEENMFWAGVVFPDMYPWTSSLPPHVKYKIRMDIDVVEKTNKIKDRYWDSGPRADPVEDFRYIWGGFAYLQDMVEQGITRSQVQAEAPVGIYLQQMPYPCFVDDSFMIILNRCFPIFMVLAWIYSVSMTVKSIVLEKELRLKETLKNQGVSNAVIWCTWFLDSFSIMSMSIFLLTIFIMHGRILHYSDPFILFLFLLAFSTATIMLCFLLSTFFSKASLAAACSGVIYFTLYLPHILCFAWQDRMTAELKKAVSLLSPVAFGFGTEYLVRFEEQGLGLQWSNIGNSPTEGDEFSFLLSMQMMLLDAAVYGLLAWYLDQVFPGDYGTPLPWYFLLQESYWLGGEGCSTREERALEKTEPLTEETEDPEHPEGIHDSFFEREHPGWVPGVCVKNLVKIFEPCGRPAVDRLNITFYENQITAFLGHNGAGKTTTLSILTGLLPPTSGTVLVGGRDIETSLDAVRQSLGMCPQHNILFHHLTVAEHMLFYAQLKGKSQEEAQLEMEAMLEDTGLHHKRNEEAQDLSGGMQRKLSVAIAFVGDAKVVILDEPTSGVDPYSRRSIWDLLLKYRSGRTIIMSTHHMDEADLLGDRIAIIAQGRLYCSGTPLFLKNCFGTGLYLTLVRKMKNIQSQRKGSEGTCSCSSKGFSTTCPAHVDDLTPEQVLDGDVNELMDVVLHHVPEAKLVECIGQELIFLLPNKNFKHRAYASLFRELEETLADLGLSSFGISDTPLEEIFLKVTEDS

SEQ ID NO: 38 - protein, 1301 aa, synthetic construct
MGFVRQIQLLLWKNWTLRKRQKIRFVVELVWPLSLFLVLIWLRNANPLYSHHECHFPNKAMPSAGMLPWLQGIFCNVNNPCFQSPTPGESPGIVSNYNNSILARVYRDFQELLMNAPESQHLGRIWTELHILSQFMDTLRTHPERIAGRGIRIRDILKDEETLTLFLIKNIGLSDSVVYLLINSQVRPEQFAHGVPDLALKDIACSEALLERFIIFSQRRGAKTVRYALCSLSQGTLQWIEDTLYANVDFFKLFRVLPTLLDSRSQGINLRSWGGILSDMSPRIQEFIHRPSMQDLLWVTRPLMQNGGPETFTKLMGILSDLLCGYPEGGGSRVLSFNWYEDNNYKAFLGIDSTRKDPIYSYDRRTTSFCNALIQSLESNPLTKIAWRAAKPLLMGKILYTPDSPAARRILKNANSTFEELEHVRKLVKAWEEVGPQIWYFFDNSTQMNMIRDTLGNPTVKDFLNRQLGEEGITAEAILNFLYKGPRESQADDMANFDWRDIFNITDRTLRLVNQYLECLVLDKFESYNDETQLTQRALSLLEENMFWAGVVFPDMYPWTSSLPPHVKYKIRMDIDVVEKTNKIKDRYWDSGPRADPVEDFRYIWGGFAYLQDMVEQGITRSQVQAEAPVGIYLQQMPYPCFVDDSFMIILNRCFPIFMVLAWIYSVSMTVKSIVLEKELRLKETLKNQGVSNAVIWCTWFLDSFSIMSMSIFLLTIFIMHGRILHYSDPFILFLFLLAFSTATIMLCFLLSTFFSKASLAAACSGVIYFTLYLPHILCFAWQDRMTAELKKAVSLLSPVAFGFGTEYLVRFEEQGLGLQWSNIGNSPTEGDEFSFLLSMQMMLLDAAVYGLLAWYLDQVFPGDYGTPLPWYFLLQESYWLGGEGCSTREERALEKTEPLTEETEDPEHPEGIHDSFFEREHPGWVPGVCVKNLVKIFEPCGRPAVDRLNITFYENQITAFLGHNGAGKTTTLSILTGLLPPTSGTVLVGGRDIETSLDAVRQSLGMCPQHNILFHHLTVAEHMLFYAQLKGKSQEEAQLEMEAMLEDTGLHHKRNEEAQDLSGGMQRKLSVAIAFVGDAKVVILDEPTSGVDPYSRRSIWDLLLKYRSGRTIIMSTHHMDEADLLGDRIAIIAQGRLYCSGTPLFLKNCFGTGLYLTLVRKMKNIQSQRKGSEGTCSCSSKGFSTTCPAHVDDLTPEQVLDGDVNELMDVVLHHVPEAKLVECIGQELIFLLPNKNFKHRAYASLFRELEETLADLGLSSFGISDTPLEEIFLKVTEDSTESHDLPLHPRAAGASRQAQD

SEQ ID NO: 39 - protein, 925 aa, synthetic construct
MGFVRQIQLLLWKNWTLRKRSHKDFLAQIVLPATFVFLALMLSIVIPPFGEYPALTLHPWIYGQQYTFFSMDEPGSEQFTVLADVLLNKPGFGNRCLKEGWLPEYPCGNSTPWKTPSVSPNITQLFQKQKWTQVNPSPSCRCSTREKLTMLPECPEGAGGLPPPQRTQRSTEILQDLTDRNISDFLVKTYPALIRSSLKSKFWVNEQRYGGISIGGKLPVVPITGEALVGFLSDLGRIMNVSGGPITREASKEIPDFLKHLETEDNIKVWFNNKGWHALVSFLNVAHNAILRASLPKDRSPEEYGITVISQPLNLTKEQLSEITVLTTSVDAVVAICVIFSMSFVPASFVLYLIQERVNKSKHLQFISGVSPTTYWVTNFLWDIMNYSVSAGLVVGIFIGFQKKAYTSPENLPALVALLLLYGWAVIPMMYPASFLFDVPSTAYVALSCANLFIGINSSAITFILELFENNRTLLRFNAVLRKLLIVFPHFCLGRGLIDLALSQAVTDVYARFGEEHSANPFHWDLIGKNLFAMVVEGVVYFLLTLLVQRHFFLSQWIAEPTKEPIVDEDDDVAEERQRIITGGNKTDILRLHELTKIYPGTSSPAVDRLCVGVRPGECFGLLGVNGAGKTTTFKMLTGDTTVTSGDATVAGKSILTNISEVHQNMGYCPQFDAIDELLTGREHLYLYARLRGVPAEEIEKVANWSIKSLGLTVYADCLAGTYSGGNKRKLSTAIALIGCPPLVLLDEPTTGMDPQARRMLWNVIVSIIREGRAVVLTSHSMEECEALCTRLAIMVKGAFRCMGTIQHLKSKFGDGYIVTMKIKSPKDDLLPDLNPVEQFFQGNFPGSVQRERHYNMLQFQVSSSSLARIFQLLLSHKDSLLIEEYSVTQTTLDQVFVNFAKQQTESHDLPLHPRAAGASRQAQD

SEQ ID NO: 40 - DNA, 3480 bp, synthetic construct
  source 1..3480: mol_type = other DNA
atgggattcgtgcggcagatccagcttctgctctggaagaattggaccctgcgtaaacggcagaagattagatttgtggtggagctggtgtggcctctgagcctgttcttggtgctgatctggctgcgaaacgccaaccctctgtactcccaccatgagtgtcacttccctaacaaggccatgccttctgctggcatgctgccttggctgcagggcatcttctgcaacgtgaacaacccctgcttccagagccccacccctggagagtctcccggcatcgtcagtaactacaacaactccatcctcgccagagtgtacagagatttccaggagctgctgatgaacgcccctgagtctcaacacctggggagaatctggaccgagctccatatactgtcacagttcatggataccctacggacccaccccgaacggatcgccggcagaggcattagaatccgggatatccttaaggacgaagagacactgactctttttctgattaagaatatcggattgtctgattcggtggtgtacctgctgatcaacagccaggtgagacctgagcagttcgcccacggcgtgcctgacttagcgctgaaggacattgcctgctctgaggccttgctggaaagattcatcatcttctctcagcggcggggggccaagacagttcggtacgccctgtgcagcctgagccagggcaccttgcagtggatcgaagacaccctgtatgctaacgtggacttctttaaactgtttagagtgttgccaaccttactggacagccggagccagggcatcaacctgagatcctggggtggaatcctgagcgatatgagccccagaatccaggagttcatccaccggcctagcatgcaggacttgctgtgggtgactcgtcccctgatgcaaaacggaggaccagaaacatttacaaagcttatgggcatcctgagcgacctcttgtgcggctaccctgagggcggcggcagccgggtgttaagctttaactggtacgaggacaacaactacaaggccttccttggtatcgatagcacacgaaaggacccaatctacagctacgaccgtagaacaaccagtttctgcaacgccctgatccagtcccttgaatctaatcctttgacaaagatcgcttggcgggccgccaagcctctgctgatgggcaagatcctgtacacccctgacagccctgccgccagaagaatcctaaagaatgccaacagcactttcgaggaactcgaacacgtgcggaagctggtcaaagcctgggaggaggtgggccctcaaatctggtacttcttcgataactccacccagatgaacatgatcagagacaccttgggaaatccgaccgtgaaggacttcctgaatagacagctaggtgaggagggaatcaccgccgaggccatcctgaactttctgtacaaaggccctcgggagtcccaggctgatgacatggccaattttgactggagagacatattcaacatcacagaccgtacccttagactggtgaaccagtacctggaatgcttagtcctggataagttcgaaagctacaacgacgagacccagctgacccaacgggcactgtctctactggaggagaatatgttctgggccggtgtggtgttccctgacatgtacccctggacaagcagcctgccacctcacgtgaaatacaagatccggatggacattgacgtggtggaaaagacaaacaagatcaaggacagatactgggacagcggacctagggccgatcctgtggaggatttccggtacatctggggtggcttcgcttacctgcaggacatggtggaacagggcatcacgagaagccaggtgcaggctgaggcccctgtgggaatctacctccaacagatgccctacccctgcttcgtggacgacagcttcatgatcatcctgaatagatgtttcccaatcttcatggtgctggcctggatctacagcgtgtccatgactgtgaagtccatcgtgctggagaaggagctgcggctaaaagagactctgaagaatcagggcgtgagcaacgccgtaatctggtgcacctggttcctggactccttctccatcatgagcatgagcatcttcctactgacaatctttatcatgcacggcagaattctgcactacagcgaccctttcatcctgtttctttttttgctggctttcagcaccgccaccatcatgctgtgcttcctgttaagcaccttcttctcaaaggccagcctagctgcagcatgctccggcgtcatctactttactttatacctgccccacatcctgtgtttcgcctggcaggacagaatgacagccgagctgaaaaaggccgtatccctgttgagccccgtggccttcgggtttggaaccgagtacctggtacggttcgaggaacaaggcctgggcctgcagtggtccaacatcggcaactcgccgaccgagggcgacgaattcagcttcctgctgtccatgcagatgatgctgctggatgccgcagtgtatggcctcctggcttggtacttggaccaggtgttccccggcgactacgggactccactgccatggtactttctgctgcaggagagctactggctgggcggcgagggctgcagcaccagagaggaaagagccctggagaagacagagcctctgactgaagaaaccgaagaccctgagcaccctgaggggatacacgactcttttttcgagagggaacatcctggatgggtccctggcgtttgcgtgaagaacctggtgaagatcttcgagccttgtggcaggccagccgtggatagactgaatatcaccttctacgagaaccagatcaccgccttcctgggccacaacggcgcgggaaagaccacaactctgagcatcctgaccggactgctgcctccaacttccggcaccgtgctcgtcggcggcagggacatcgagaccagtctggacgccgtgagacagagcctcggcatgtgccctcagcacaatatcctgtttcaccacttaaccgttgcagaacacatgctgttctacgcccagttaaaaggcaagtcgcaggaggaggcccagctggagatggaagcaatgctcgaagatacaggcctgcaccataagagaaacgaagaggcccaggatctctccggcggcatgcagagaaaactgagcgtagccatcgccttcgtgggagatgcaaaggtggtaatcctagatgagcctacatctggggtggacccgtacagccggcgcagtatttgggatttactgctgaagtacagaagcggtagaaccatcatcatgtctacccaccacatggacgaggctgatctgctgggagatcggatcgccataatcgcccagggaagactgtattgcagcggcacaccactgttcctcaaaaactgctttgggacgggactgtacctgacgctggtc

SEQ ID NO: 41 - DNA, 3660 bp, synthetic construct
  source 1..3660: mol_type = other DNA
atgggattcgtgcggcagatccagcttctgctctggaagaattggaccctgcgtaaacggcagaagattagatttgtggtggagctggtgtggcctctgagcctgttcttggtgctgatctggctgcgaaacgccaaccctctgtactcccaccatgagtgtcacttccctaacaaggccatgccttctgctggcatgctgccttggctgcagggcatcttctgcaacgtgaacaacccctgcttccagagccccacccctggagagtctcccggcatcgtcagtaactacaacaactccatcctcgccagagtgtacagagatttccaggagctgctgatgaacgcccctgagtctcaacacctggggagaatctggaccgagctccatatactgtcacagttcatggataccctacggacccaccccgaacggatcgccggcagaggcattagaatccgggatatccttaaggacgaagagacactgactctttttctgattaagaatatcggattgtctgattcggtggtgtacctgctgatcaacagccaggtgagacctgagcagttcgcccacggcgtgcctgacttagcgctgaaggacattgcctgctctgaggccttgctggaaagattcatcatcttctctcagcggcggggggccaagacagttcggtacgccctgtgcagcctgagccagggcaccttgcagtggatcgaagacaccctgtatgctaacgtggacttctttaaactgtttagagtgttgccaaccttactggacagccggagccagggcatcaacctgagatcctggggtggaatcctgagcgatatgagccccagaatccaggagttcatccaccggcctagcatgcaggacttgctgtgggtgactcgtcccctgatgcaaaacggaggaccagaaacatttacaaagcttatgggcatcctgagcgacctcttgtgcggctaccctgagggcggcggcagccgggtgttaagctttaactggtacgaggacaacaactacaaggccttccttggtatcgatagcacacgaaaggacccaatctacagctacgaccgtagaacaaccagtttctgcaacgccctgatccagtcccttgaatctaatcctttgacaaagatcgcttggcgggccgccaagcctctgctgatgggcaagatcctgtacacccctgacagccctgccgccagaagaatcctaaagaatgccaacagcactttcgaggaactcgaacacgtgcggaagctggtcaaagcctgggaggaggtgggccctcaaatctggtacttcttcgataactccacccagatgaacatgatcagagacaccttgggaaatccgaccgtgaaggacttcctgaatagacagctaggtgaggagggaatcaccgccgaggccatcctgaactttctgtacaaaggccctcgggagtcccaggctgatgacatggccaattttgactggagagacatattcaacatcacagaccgtacccttagactggtgaaccagtacctggaatgcttagtcctggataagttcgaaagctacaacgacgagacccagctgacccaacgggcactgtctctactggaggagaatatgttctgggccggtgtggtgttccctgacatgtacccctggacaagcagcctgccacctcacgtgaaatacaagatccggatggacattgacgtggtggaaaagacaaacaagatcaaggacagatactgggacagcggacctagggccgatcctgtggaggatttccggtacatctggggtggcttcgcttacctgcaggacatggtggaacagggcatcacgagaagccaggtgcaggctgaggcccctgtgggaatctacctccaacagatgccctacccctgcttcgtggacgacagcttcatgatcatcctgaatagatgtttcccaatcttcatggtgctggcctggatctacagcgtgtccatgactgtgaagtccatcgtgctggagaaggagctgcggctaaaagagactctgaagaatcagggcgtgagcaacgccgtaatctggtgcacctggttcctggactccttctccatcatgagcatgagcatcttcctactgacaatctttatcatgcacggcagaattctgcactacagcgaccctttcatcctgtttctttttttgctggctttcagcaccgccaccatcatgctgtgcttcctgttaagcaccttcttctcaaaggccagcctagctgcagcatgctccggcgtcatctactttactttatacctgccccacatcctgtgtttcgcctggcaggacagaatgacagccgagctgaaaaaggccgtatccctgttgagccccgtggccttcgggtttggaaccgagtacctggtacggttcgaggaacaaggcctgggcctgcagtggtccaacatcggcaactcgccgaccgagggcgacgaattcagcttcctgctgtccatgcagatgatgctgctggatgccgcagtgtatggcctcctggcttggtacttggaccaggtgttccccggcgactacgggactccactgccatggtactttctgctgcaggagagctactggctgggcggcgagggctgcagcaccagagaggaaagagccctggagaagacagagcctctgactgaagaaaccgaagaccctgagcaccctgaggggatacacgactcttttttcgagagggaacatcctggatgggtccctggcgtttgcgtgaagaacctggtgaagatcttcgagccttgtggcaggccagccgtggatagactgaatatcaccttctacgagaaccagatcaccgccttcctgggccacaacggcgcgggaaagaccacaactctgagcatcctgaccggactgctgcctccaacttccggcaccgtgctcgtcggcggcagggacatcgagaccagtctggacgccgtgagacagagcctcggcatgtgccctcagcacaatatcctgtttcaccacttaaccgttgcagaacacatgctgttctacgcccagttaaaaggcaagtcgcaggaggaggcccagctggagatggaagcaatgctcgaagatacaggcctgcaccataagagaaacgaagaggcccaggatctctccggcggcatgcagagaaaactgagcgtagccatcgccttcgtgggagatgcaaaggtggtaatcctagatgagcctacatctggggtggacccgtacagccggcgcagtatttgggatttactgctgaagtacagaagcggtagaaccatcatcatgtctacccaccacatggacgaggctgatctgctgggagatcggatcgccataatcgcccagggaagactgtattgcagcggcacaccactgttcctcaaaaactgctttgggacgggactgtacctgacgctggtccggaaaatgaagaacatccagtcccagagaaagggctctgaagggacctgttcttgcagctctaagggcttcagtaccacctgccctgcccacgtggacgacctgactcccgaacaggtgctggacggcgatgtgaacgagctgatggacgtggtgctgcatcacgtacccgaagccaag

SEQ ID NO: 42 - DNA, 3840 bp, synthetic construct
  source 1..3840: mol_type = other DNA
atgggattcgtgcggcagatccagcttctgctctggaagaattggaccctgcgtaaacggcagaagattagatttgtggtggagctggtgtggcctctgagcctgttcttggtgctgatctggctgcgaaacgccaaccctctgtactcccaccatgagtgtcacttccctaacaaggccatgccttctgctggcatgctgccttggctgcagggcatcttctgcaacgtgaacaacccctgcttccagagccccacccctggagagtctcccggcatcgtcagtaactacaacaactccatcctcgccagagtgtacagagatttccaggagctgctgatgaacgcccctgagtctcaacacctggggagaatctggaccgagctccatatactgtcacagttcatggataccctacggacccaccccgaacggatcgccggcagaggcattagaatccgggatatccttaaggacgaagagacactgactctttttctgattaagaatatcggattgtctgattcggtggtgtacctgctgatcaacagccaggtgagacctgagcagttcgcccacggcgtgcctgacttagcgctgaaggacattgcctgctctgaggccttgctggaaagattcatcatcttctctcagcggcggggggccaagacagttcggtacgccctgtgcagcctgagccagggcaccttgcagtggatcgaagacaccctgtatgctaacgtggacttctttaaactgtttagagtgttgccaaccttactggacagccggagccagggcatcaacctgagatcctggggtggaatcctgagcgatatgagccccagaatccaggagttcatccaccggcctagcatgcaggacttgctgtgggtgactcgtcccctgatgcaaaacggaggaccagaaacatttacaaagcttatgggcatcctgagcgacctcttgtgcggctaccctgagggcggcggcagccgggtgttaagctttaactggtacgaggacaacaactacaaggccttccttggtatcgatagcacacgaaaggacccaatctacagctacgaccgtagaacaaccagtttctgcaacgccctgatccagtcccttgaatctaatcctttgacaaagatcgcttggcgggccgccaagcctctgctgatgggcaagatcctgtacacccctgacagccctgccgccagaagaatcctaaagaatgccaacagcactttcgaggaactcgaacacgtgcggaagctggtcaaagcctgggaggaggtgggccctcaaatctggtacttcttcgataactccacccagatgaacatgatcagagacaccttgggaaatccgaccgtgaaggacttcctgaatagacagctaggtgaggagggaatcaccgccgaggccatcctgaactttctgtacaaaggccctcgggagtcccaggctgatgacatggccaattttgactggagagacatattcaacatcacagaccgtacccttagactggtgaaccagtacctggaatgcttagtcctggataagttcgaaagctacaacgacgagacccagctgacccaacgggcactgtctctactggaggagaatatgttctgggccggtgtggtgttccctgacatgtacccctggacaagcagcctgccacctcacgtgaaatacaagatccggatggacattgacgtggtggaaaagacaaacaagatcaaggacagatactgggacagcggacctagggccgatcctgtggaggatttccggtacatctggggtggcttcgcttacctgcaggacatggtggaacagggcatcacgagaagccaggtgcaggctgaggcccctgtgggaatctacctccaacagatgccctacccctgcttcgtggacgacagcttcatgatcatcctgaatagatgtttcccaatcttcatggtgctggcctggatctacagcgtgtccatgactgtgaagtccatcgtgctggagaaggagctgcggctaaaagagactctgaagaatcagggcgtgagcaacgccgtaatctggtgcacctggttcctggactccttctccatcatgagcatgagcatcttcctactgacaatctttatcatgcacggcagaattctgcactacagcgaccctttcatcctgtttctttttttgctggctttcagcaccgccaccatcatgctgtgcttcctgttaagcaccttcttctcaaaggccagcctagctgcagcatgctccggcgtcatctactttactttatacctgccccacatcctgtgtttcgcctggcaggacagaatgacagccgagctgaaaaaggccgtatccctgttgagccccgtggccttcgggtttggaaccgagtacctggtacggttcgaggaacaaggcctgggcctgcagtggtccaacatcggcaactcgccgaccgagggcgacgaattcagcttcctgctgtccatgcagatgatgctgctggatgccgcagtgtatggcctcctggcttggtacttggaccaggtgttccccggcgactacgggactccactgccatggtactttctgctgcaggagagctactggctgggcggcgagggctgcagcaccagagaggaaagagccctggagaagacagagcctctgactgaagaaaccgaagaccctgagcaccctgaggggatacacgactcttttttcgagagggaacatcctggatgggtccctggcgtttgcgtgaagaacctggtgaagatcttcgagccttgtggcaggccagccgtggatagactgaatatcaccttctacgagaaccagatcaccgccttcctgggccacaacggcgcgggaaagaccacaactctgagcatcctgaccggactgctgcctccaacttccggcaccgtgctcgtcggcggcagggacatcgagaccagtctggacgccgtgagacagagcctcggcatgtgccctcagcacaatatcctgtttcaccacttaaccgttgcagaacacatgctgttctacgcccagttaaaaggcaagtcgcaggaggaggcccagctggagatggaagcaatgctcgaagatacaggcctgcaccataagagaaacgaagaggcccaggatctctccggcggcatgcagagaaaactgagcgtagccatcgccttcgtgggagatgcaaaggtggtaatcctagatgagcctacatctggggtggacccgtacagccggcgcagtatttgggatttactgctgaagtacagaagcggtagaaccatcatcatgtctacccaccacatggacgaggctgatctgctgggagatcggatcgccataatcgcccagggaagactgtattgcagcggcacaccactgttcctcaaaaactgctttgggacgggactgtacctgacgctggtccggaaaatgaagaacatccagtcccagagaaagggctctgaagggacctgttcttgcagctctaagggcttcagtaccacctgccctgcccacgtggacgacctgactcccgaacaggtgctggacggcgatgtgaacgagctgatggacgtggtgctgcatcacgtacccgaagccaagctggttgaatgcatcggccaggagctcattttccttcttcctaacaagaacttcaagcacagagcttatgcctctctgttcagggaactggaggaaaccctagccgacctgggtctgtctagcttcggcatctctgacacacctctggaggagatctttctgaaagtgactgaggattct

SEQ ID NO: 43 - DNA, 3903 bp, synthetic construct
  source 1..3903: mol_type = other DNA
atgggattcgtgcggcagatccagcttctgctctggaagaattggaccctgcgtaaacggcagaagattagatttgtggtggagctggtgtggcctctgagcctgttcttggtgctgatctggctgcgaaacgccaaccctctgtactcccaccatgagtgtcacttccctaacaaggccatgccttctgctggcatgctgccttggctgcagggcatcttctgcaacgtgaacaacccctgcttccagagccccacccctggagagtctcccggcatcgtcagtaactacaacaactccatcctcgccagagtgtacagagatttccaggagctgctgatgaacgcccctgagtctcaacacctggggagaatctggaccgagctccatatactgtcacagttcatggataccctacggacccaccccgaacggatcgccggcagaggcattagaatccgggatatccttaaggacgaagagacactgactctttttctgattaagaatatcggattgtctgattcggtggtgtacctgctgatcaacagccaggtgagacctgagcagttcgcccacggcgtgcctgacttagcgctgaaggacattgcctgctctgaggccttgctggaaagattcatcatcttctctcagcggcggggggccaagacagttcggtacgccctgtgcagcctgagccagggcaccttgcagtggatcgaagacaccctgtatgctaacgtggacttctttaaactgtttagagtgttgccaaccttactggacagccggagccagggcatcaacctgagatcctggggtggaatcctgagcgatatgagccccagaatccaggagttcatccaccggcctagcatgcaggacttgctgtgggtgactcgtcccctgatgcaaaacggaggaccagaaacatttacaaagcttatgggcatcctgagcgacctcttgtgcggctaccctgagggcggcggcagccgggtgttaagctttaactggtacgaggacaacaactacaaggccttccttggtatcgatagcacacgaaaggacccaatctacagctacgaccgtagaacaaccagtttctgcaacgccctgatccagtcccttgaatctaatcctttgacaaagatcgcttggcgggccgccaagcctctgctgatgggcaagatcctgtacacccctgacagccctgccgccagaagaatcctaaagaatgccaacagcactttcgaggaactcgaacacgtgcggaagctggtcaaagcctgggaggaggtgggccctcaaatctggtacttcttcgataactccacccagatgaacatgatcagagacaccttgggaaatccgaccgtgaaggacttcctgaatagacagctaggtgaggagggaatcaccgccgaggccatcctgaactttctgtacaaaggccctcgggagtcccaggctgatgacatggccaattttgactggagagacatattcaacatcacagaccgtacccttagactggtgaaccagtacctggaatgcttagtcctggataagttcgaaagctacaacgacgagacccagctgacccaacgggcactgtctctactggaggagaatatgttctgggccggtgtggtgttccctgacatgtacccctggacaagcagcctgccacctcacgtgaaatacaagatccggatggacattgacgtggtggaaaagacaaacaagatcaaggacagatactgggacagcggacctagggccgatcctgtggaggatttccggtacatctggggtggcttcgcttacctgcaggacatggtggaacagggcatcacgagaagccaggtgcaggctgaggcccctgtgggaatctacctccaacagatgccctacccctgcttcgtggacgacagcttcatgatcatcctgaatagatgtttcccaatcttcatggtgctggcctggatctacagcgtgtccatgactgtgaagtccatcgtgctggagaaggagctgcggctaaaagagactctgaagaatcagggcgtgagcaacgccgtaatctggtgcacctggttcctggactccttctccatcatgagcatgagcatcttcctactgacaatctttatcatgcacggcagaattctgcactacagcgaccctttcatcctgtttctttttttgctggctttcagcaccgccaccatcatgctgtgcttcctgttaagcaccttcttctcaaaggccagcctagctgcagcatgctccggcgtcatctactttactttatacctgccccacatcctgtgtttcgcctggcaggacagaatgacagccgagctgaaaaaggccgtatccctgttgagccccgtggccttcgggtttggaaccgagtacctggtacggttcgaggaacaaggcctgggcctgcagtggtccaacatcggcaactcgccgaccgagggcgacgaattcagcttcctgctgtccatgcagatgatgctgctggatgccgcagtgtatggcctcctggcttggtacttggaccaggtgttccccggcgactacgggactccactgccatggtactttctgctgcaggagagctactggctgggcggcgagggctgcagcaccagagaggaaagagccctggagaagacagagcctctgactgaagaaaccgaagaccctgagcaccctgaggggatacacgactcttttttcgagagggaacatcctggatgggtccctggcgtttgcgtgaagaacctggtgaagatcttcgagccttgtggcaggccagccgtggatagactgaatatcaccttctacgagaaccagatcaccgccttcctgggccacaacggcgcgggaaagaccacaactctgagcatcctgaccggactgctgcctccaacttccggcaccgtgctcgtcggcggcagggacatcgagaccagtctggacgccgtgagacagagcctcggcatgtgccctcagcacaatatcctgtttcaccacttaaccgttgcagaacacatgctgttctacgcccagttaaaaggcaagtcgcaggaggaggcccagctggagatggaagcaatgctcgaagatacaggcctgcaccataagagaaacgaagaggcccaggatctctccggcggcatgcagagaaaactgagcgtagccatcgccttcgtgggagatgcaaaggtggtaatcctagatgagcctacatctggggtggacccgtacagccggcgcagtatttgggatttactgctgaagtacagaagcggtagaaccatcatcatgtctacccaccacatggacgaggctgatctgctgggagatcggatcgccataatcgcccagggaagactgtattgcagcggcacaccactgttcctcaaaaactgctttgggacgggactgtacctgacgctggtccggaaaatgaagaacatccagtcccagagaaagggctctgaagggacctgttcttgcagctctaagggcttcagtaccacctgccctgcccacgtggacgacctgactcccgaacaggtgctggacggcgatgtgaacgagctgatggacgtggtgctgcatcacgtacccgaagccaagctggttgaatgcatcggccaggagctcattttccttcttcctaacaagaacttcaagcacagagcttatgcctctctgttcagggaactggaggaaaccctagccgacctgggtctgtctagcttcggcatctctgacacacctctggaggagatctttctgaaagtgactgaggattctaccgagagccatgatctgcctcttcacccacgagctgccggcgccagcagacaggcccaggac

SEQ ID NO: 44 - DNA, 2775 bp, synthetic construct
  source 1..2775: mol_type = other DNA
atgggattcgtgcggcagatccagcttctgctctggaagaattggaccctgcgtaaacggagtcataaagacttcctcgctcagatcgtgctcccggctacattcgtgtttctggccctcatgctgtctatcgtgatcccacctttcggcgaataccctgcgctgaccctgcacccctggatatacggtcagcaatacacctttttcagcatggacgagcccggaagcgagcagttcaccgtgctggccgatgtgctgctgaacaagcctggcttcggcaaccggtgcctgaaagaaggatggctgccagagtacccctgcggcaatagcacaccttggaagacccctagcgtgtcccctaacatcacccagctgtttcaaaaacagaaatggacccaagtgaatccttcaccttcatgcagatgttctacacgtgaaaagctgaccatgttacccgagtgtcctgaaggagctggcggccttcctcctccccagaggacccagagaagcaccgaaatcctgcaggacctgacagaccggaacatctccgactttcttgtcaagacctaccctgccctgattaggagtagcctgaaatctaagttttgggttaatgaacagcggtacggcggcatcagcatcggcggtaagctgcccgtggtgcctattacaggcgaggccctggtgggcttcctcagtgatttgggacggataatgaacgtgagtggcggcccaatcacacgggaagccagcaaagagatccctgatttcctgaagcacctggaaacagaggataatataaaggtgtggttcaacaacaaaggctggcacgccctggtgagtttcctcaacgtagcccacaacgctatcctgagagcctctctacctaaggacagaagccccgaagagtacggcattaccgtgatcagccagcccctaaacctgacaaaggaacagctgagcgagattaccgtcctgacaacctccgttgacgcggtggtggcgatctgcgtgatcttttctatgagcttcgtgcctgccagcttcgtgctgtacctgatccaggagagagtgaacaagagcaagcacctgcaatttatttctggcgtgagcccaaccacctactgggtgaccaacttcctgtgggacatcatgaactacagcgtgtctgccggcctggtggtaggcatcttcatcggcttccagaagaaggcctacacctctcctgagaatctgcctgctctcgtggccctgctgctgctgtacggctgggccgtgatccccatgatgtaccccgctagcttcttatttgacgtgccctcaacagcatacgtggccttatcctgcgccaacctgtttataggaatcaattctagcgccatcacgttcatcctagaactgttcgagaacaaccggacactgctgcgattcaacgccgtcctgcggaagctcctgattgtgttccctcatttctgtctgggcagagggctgatcgacctggccctgagccaagccgtgaccgatgtgtacgcgagattcggcgaggagcactccgccaaccctttccactgggacctgatcggcaagaatctgttcgccatggttgtggagggtgtggtgtacttcctgcttacactgctggtgcagagacacttcttcctgtcccagtggattgccgaacccaccaaggaacccatcgtcgacgaggatgacgacgtggccgaggagagacagagaatcatcaccggcgggaacaaaaccgacatcctgagactccacgagctgacaaagatctatcctggcacaagcagccccgccgtggatcggctgtgtgtgggcgtcagacctggcgagtgcttcggcctgctgggcgtgaacggcgccggcaagaccacaaccttcaagatgctgaccggcgacaccacggtgacctccggcgacgccacagtggccggcaaaagcatcctcacaaacatctccgaagtgcaccagaacatgggctactgcccccagtttgatgctatagacgagctgttgaccggtagagaacacctgtacctgtacgccagactgagaggcgtgcctgctgaagagatcgaaaaggtggcaaactggagcatcaagtcactgggcctgacagtctacgccgactgcctggccggcacgtactctggcggcaataagcggaaactgagcaccgccattgccttgattggatgtccgcctctggtgctgctggacgagccgacaacaggcatggacccccaagcccggagaatgctgtggaacgtgatcgtgagcataatcagagagggcagagccgtggttttgacttctcacagcatggaagaatgtgaagcgctctgcacccggcttgccatcatggtcaaaggcgccttccggtgcatgggcaccattcagcacctgaagtccaagttcggcgacggctacatcgtgacaatgaagatcaaatctcccaaggacgacctgcttccagatctgaaccctgtggaacagttcttccagggaaatttccctggaagcgtgcagagagagagacactacaatatgctgcagtttcaggtaagcagcagcagccttgctcggatctttcagctgctgcttagccacaaggactctctgctgatcgaagagtacagcgtgacccagacaacgcttgatcaggtgttcgtgaacttcgccaagcagcaaaccgagagccatgatctgcctcttcacccacgagctgccggcgccagcagacaggcccaggac